European Patent Application EP 4 253 544 A2, published October 4, 2023. Title: MODIFIED MESSENGER RNA COMPRISING FUNCTIONAL RNA ELEMENTS. Applicant: MODERNATX, INC. Application US. The sequence listing filed with the application follows.

SEQUENCE LISTING (535 sequences)

SEQ ID NO: 1 - skipped

SEQ ID NO: 2 - RNA, 10 nt, synthetic construct
  misc_feature 1..10: note = V1
  source 1..10: mol_type = other RNA
ccccggcgcc

SEQ ID NO: 3 - skipped

SEQ ID NO: 4 - RNA, 20 nt, synthetic construct
  misc_feature 1..20: note = CG1
  source 1..20: mol_type = other RNA
gcgccccgcggcgccccgcg

SEQ ID NO: 5 - RNA, 20 nt, synthetic construct
  misc_feature 1..20: note = CG2
  source 1..20: mol_type = other RNA
cccgcccgccccgccccgcc

SEQ ID NO: 6 - RNA, 10 nt, synthetic construct
  misc_feature 1..10: note = GC Scramble #1
  source 1..10: mol_type = other RNA
ggggcgcccg

SEQ ID NO: 7 - RNA, 10 nt, synthetic construct
  misc_feature 1..10: note = GC Scramble #2
  source 1..10: mol_type = other RNA
gcccgcccgc

SEQ ID NO: 8 - RNA, 10 nt, synthetic construct
  misc_feature 1..10: note = GC Scramble #3
  source 1..10: mol_type = other RNA
gcgccccgcg

SEQ ID NO: 9-12 - skipped (4 entries)

SEQ ID NO: 13 - RNA, 12 nt, synthetic construct
  misc_feature 1..12: note = (CCG)4
  source 1..12: mol_type = other RNA
ccgccgccgccg

SEQ ID NO: 14 - RNA, 15 nt, synthetic construct
  misc_feature 1..15: note = (CCG)5
  source 1..15: mol_type = other RNA
ccgccgccgccgccg

SEQ ID NO: 15 - RNA, 18 nt, synthetic construct
  misc_feature 1..18: note = (CCG)6
  source 1..18: mol_type = other RNA
ccgccgccgccgccgccg

SEQ ID NO: 16 - RNA, 21 nt, synthetic construct
  misc_feature 1..21: note = (CCG)7
  source 1..21: mol_type = other RNA
ccgccgccgccgccgccgccg

SEQ ID NO: 17 - RNA, 24 nt, synthetic construct
  misc_feature 1..24: note = (CCG)8
  source 1..24: mol_type = other RNA
ccgccgccgccgccgccgccgccg

SEQ ID NO: 18 - RNA, 27 nt, synthetic construct
  misc_feature 1..27: note = (CCG)9
  source 1..27: mol_type = other RNA
ccgccgccgccgccgccgccgccgccg

SEQ ID NO: 19 - RNA, 30 nt, synthetic construct
  misc_feature 1..30: note = (CCG)10
  source 1..30: mol_type = other RNA
ccgccgccgccgccgccgccgccgccgccg

SEQ ID NO: 20 - skipped

SEQ ID NO: 21 - RNA, 12 nt, synthetic construct
  misc_feature 1..12: note = (GCC)4
  source 1..12: mol_type = other RNA
gccgccgccgcc

SEQ ID NO: 22 - RNA, 15 nt, synthetic construct
  misc_feature 1..15: note = (GCC)5
  source 1..15: mol_type = other RNA
gccgccgccgccgcc

SEQ ID NO: 23 - RNA, 18 nt, synthetic construct
  misc_feature 1..18: note = (GCC)6
  source 1..18: mol_type = other RNA
gccgccgccgccgccgcc

SEQ ID NO: 24 - RNA, 21 nt, synthetic construct
  misc_feature 1..21: note = (GCC)7
  source 1..21: mol_type = other RNA
gccgccgccgccgccgccgcc

SEQ ID NO: 25 - RNA, 24 nt, synthetic construct
  misc_feature 1..24: note = (GCC)8
  source 1..24: mol_type = other RNA
gccgccgccgccgccgccgccgcc

SEQ ID NO: 26 - RNA, 27 nt, synthetic construct
  misc_feature 1..27: note = (GCC)9
  source 1..27: mol_type = other RNA
gccgccgccgccgccgccgccgccgcc

SEQ ID NO: 27 - RNA, 30 nt, synthetic construct
  misc_feature 1..30: note = (GCC)10
  source 1..30: mol_type = other RNA
gccgccgccgccgccgccgccgccgccgcc

SEQ ID NO: 28 - RNA, 16 nt, synthetic construct
  misc_feature 1..16: note = SL1
  source 1..16: mol_type = other RNA
ccgcggcgccccgcgg

SEQ ID NO: 29 - RNA, 17 nt, synthetic construct
  misc_feature 1..17: note = SL2
  source 1..17: mol_type = other RNA
gcgcgcatatagcgcgc

SEQ ID NO: 30 - RNA, 26 nt, synthetic construct
  misc_feature 1..26: note = SL3
  source 1..26: mol_type = other RNA
catggtggcggcccgccgccaccatg

SEQ ID NO: 31 - RNA, 23 nt, synthetic construct
  misc_feature 1..23: note = SL4
  source 1..23: mol_type = other RNA
catggtggcccgccgccaccatg

SEQ ID NO: 32 - RNA, 22 nt, synthetic construct
  misc_feature 1..22: note = SL5
  source 1..22: mol_type = other RNA
catggtgcccgccgccaccatg

SEQ ID NO: 33 - RNA, 47 nt, synthetic construct
  misc_feature 1..47: note = Standard UTR
  source 1..47: mol_type = other RNA
gggaaataagagagaaaagaagagtaagaagaaatataagagccacc

SEQ ID NO: 34 - RNA, 57 nt, synthetic construct
  misc_feature 1..57: note = V1-UTR
  source 1..57: mol_type = other RNA
gggaaataagagagaaaagaagagtaagaagaaatataagaccccggcgccgccacc

SEQ ID NO: 35 - RNA, 57 nt, synthetic construct
  misc_feature 1..57: note = V1-1-UTR
  source 1..57: mol_type = other RNA
gggaaataagagagaaaagaagagtaagaagaaatataagccccggcgccagccacc

SEQ ID NO: 36 - RNA, 57 nt, synthetic construct
  misc_feature 1..57: note = V1-2-UTR
  source 1..57: mol_type = other RNA
gggaaataagagagaaaagaagagtaagaagaaatataaccccggcgccgagccacc

SEQ ID NO: 37 - RNA, 57 nt, synthetic construct
  misc_feature 1..57: note = V1-3-UTR
  source 1..57: mol_type = other RNA
gggaaataagagagaaaagaagagtaagaagaaatataccccggcgccagagccacc

SEQ ID NO: 38 - RNA, 57 nt, synthetic construct
  misc_feature 1..57: note = V1-4-UTR
  source 1..57: mol_type = other RNA
gggaaataagagagaaaagaagagtaagaagaaatatccccggcgccaagagccacc

SEQ ID NO: 39 - RNA, 57 nt, synthetic construct
  misc_feature 1..57: note = V1-5-UTR
  source 1..57: mol_type = other RNA
gggaaataagagagaaaagaagagtaagaagaaataccccggcgcctaagagccacc

SEQ ID NO: 40 - RNA, 57 nt, synthetic construct
  misc_feature 1..57: note = V1-6-UTR
  source 1..57: mol_type = other RNA
gggaaataagagagaaaagaagagtaagaagaaatccccggcgccataagagccacc

SEQ ID NO: 41 - RNA, 57 nt, synthetic construct
  misc_feature 1..57: note = V1-7-UTR
  source 1..57: mol_type = other RNA
gggaaataagagagaaaagaagagtaagaagaaaccccggcgcctataagagccacc

SEQ ID NO: 42 - RNA, 57 nt, synthetic construct
  misc_feature 1..57: note = V1-8-UTR
  source 1..57: mol_type = other RNA
gggaaataagagagaaaagaagagtaagaagaaccccggcgccatataagagccacc

SEQ ID NO: 43 - RNA, 57 nt, synthetic construct
  misc_feature 1..57: note = V1-9-UTR
  source 1..57: mol_type = other RNA
gggaaataagagagaaaagaagagtaagaagaccccggcgccaatataagagccacc

SEQ ID NO: 44 - RNA, 57 nt, synthetic construct
  misc_feature 1..57: note = V1-10-UTR
  source 1..57: mol_type = other RNA
gggaaataagagagaaaagaagagtaagaagccccggcgccaaatataagagccacc

SEQ ID NO: 45 - RNA, 57 nt, synthetic construct
  misc_feature 1..57: note = V1-11-UTR
  source 1..57: mol_type = other RNA
gggaaataagagagaaaagaagagtaagaaccccggcgccgaaatataagagccacc

SEQ ID NO: 46 - RNA, 57 nt, synthetic construct
  misc_feature 1..57: note = V1-12-UTR
  source 1..57: mol_type = other RNA
gggaaataagagagaaaagaagagtaagaccccggcgccagaaatataagagccacc

SEQ ID NO: 47 - RNA, 57 nt, synthetic construct
  misc_feature 1..57: note = V1-13-UTR
  source 1..57: mol_type = other RNA
gggaaataagagagaaaagaagagtaagccccggcgccaagaaatataagagccacc

SEQ ID NO: 48 - RNA, 57 nt, synthetic construct
  misc_feature 1..57: note = V1-14-UTR
  source 1..57: mol_type = other RNA
gggaaataagagagaaaagaagagtaaccccggcgccgaagaaatataagagccacc

SEQ ID NO: 49 - RNA, 57 nt, synthetic construct
  misc_feature 1..57: note = V1-15-UTR
  source 1..57: mol_type = other RNA
gggaaataagagagaaaagaagagtaccccggcgccagaagaaatataagagccacc

SEQ ID NO: 50 - RNA, 57 nt, synthetic construct
  misc_feature 1..57: note = V1-16-UTR
  source 1..57: mol_type = other RNA
gggaaataagagagaaaagaagagtccccggcgccaagaagaaatataagagccacc

SEQ ID NO: 51 - RNA, 57 nt, synthetic construct
  misc_feature 1..57: note = V1-17-UTR
  source 1..57: mol_type = other RNA
gggaaataagagagaaaagaagagccccggcgcctaagaagaaatataagagccacc

SEQ ID NO: 52 - RNA, 57 nt, synthetic construct
  misc_feature 1..57: note = V3-UTR
  source 1..57: mol_type = other RNA
gggaaataagagagaaaagaagaccccggcgccgtaagaagaaatataagagccacc

SEQ ID NO: 53 - RNA, 57 nt, synthetic construct
  misc_feature 1..57: note = V4-UTR
  source 1..57: mol_type = other RNA
gggccccggcgccaaataagagagaaaagaagagtaagaagaaatataagagccacc

SEQ ID NO: 54 - RNA, 54 nt, synthetic construct
  misc_feature 1..54: note = V2-UTR
  source 1..54: mol_type = other RNA
gggaaataagagagaaaagaagagtaagaagaaatataagaccccggcgccacc

SEQ ID NO: 55 - RNA, 54 nt, synthetic construct
  misc_feature 1..54: note = V2-1-UTR
  source 1..54: mol_type = other RNA
gggaaataagagagaaaagaagagtaagaagaaatataagccccggcagccacc

SEQ ID NO: 56 - RNA, 54 nt, synthetic construct
  misc_feature 1..54: note = V2-2-UTR
  source 1..54: mol_type = other RNA
gggaaataagagagaaaagaagagtaagaagaaatataaccccggcgagccacc

SEQ ID NO: 57 - RNA, 54 nt, synthetic construct
  misc_feature 1..54: note = V2-3-UTR
  source 1..54: mol_type = other RNA
gggaaataagagagaaaagaagagtaagaagaaatataccccggcagagccacc

SEQ ID NO: 58 - RNA, 54 nt, synthetic construct
  misc_feature 1..54: note = V2-4-UTR
  source 1..54: mol_type = other RNA
gggaaataagagagaaaagaagagtaagaagaaatatccccggcaagagccacc

SEQ ID NO: 59 - RNA, 54 nt, synthetic construct
  misc_feature 1..54: note = V2-5-UTR
  source 1..54: mol_type = other RNA
gggaaataagagagaaaagaagagtaagaagaaataccccggctaagagccacc

SEQ ID NO: 60 - RNA, 54 nt, synthetic construct
  misc_feature 1..54: note = V2-6-UTR
  source 1..54: mol_type = other RNA
gggaaataagagagaaaagaagagtaagaagaaatccccggcataagagccacc

SEQ ID NO: 61 - RNA, 54 nt, synthetic construct
  misc_feature 1..54: note = V2-7-UTR
  source 1..54: mol_type = other RNA
gggaaataagagagaaaagaagagtaagaagaaaccccggctataagagccacc

SEQ ID NO: 62 - RNA, 54 nt, synthetic construct
  misc_feature 1..54: note = V2-8-UTR
  source 1..54: mol_type = other RNA
gggaaataagagagaaaagaagagtaagaagaaccccggcatataagagccacc

SEQ ID NO: 63 - RNA, 54 nt, synthetic construct
  misc_feature 1..54: note = V2-9-UTR
  source 1..54: mol_type = other RNA
gggaaataagagagaaaagaagagtaagaagaccccggcaatataagagccacc

SEQ ID NO: 64 - RNA, 54 nt, synthetic construct
  misc_feature 1..54: note = V2-10-UTR
  source 1..54: mol_type = other RNA
gggaaataagagagaaaagaagagtaagaagccccggcaaatataagagccacc

SEQ ID NO: 65 - RNA, 54 nt, synthetic construct
  misc_feature 1..54: note = V2-11-UTR
  source 1..54: mol_type = other RNA
gggaaataagagagaaaagaagagtaagaaccccggcgaaatataagagccacc

SEQ ID NO: 66 - RNA, 54 nt, synthetic construct
  misc_feature 1..54: note = V2-12-UTR
  source 1..54: mol_type = other RNA
gggaaataagagagaaaagaagagtaagaccccggcagaaatataagagccacc

SEQ ID NO: 67 - RNA, 54 nt, synthetic construct
  misc_feature 1..54: note = V2-13-UTR
  source 1..54: mol_type = other RNA
gggaaataagagagaaaagaagagtaagccccggcaagaaatataagagccacc

SEQ ID NO: 68 - RNA, 54 nt, synthetic construct
  misc_feature 1..54: note = V2-14-UTR
  source 1..54: mol_type = other RNA
gggaaataagagagaaaagaagagtaaccccggcgaagaaatataagagccacc

SEQ ID NO: 69 - RNA, 54 nt, synthetic construct
  misc_feature 1..54: note = V2-15-UTR
  source 1..54: mol_type = other RNA
gggaaataagagagaaaagaagagtaccccggcagaagaaatataagagccacc

SEQ ID NO: 70 - RNA, 54 nt, synthetic construct
  misc_feature 1..54: note = V2-16-UTR
  source 1..54: mol_type = other RNA
gggaaataagagagaaaagaagagtccccggcaagaagaaatataagagccacc

SEQ ID NO: 71 - RNA, 54 nt, synthetic construct
  misc_feature 1..54: note = V2-17-UTR
  source 1..54: mol_type = other RNA
gggaaataagagagaaaagaagagccccggctaagaagaaatataagagccacc

SEQ ID NO: 72 - RNA, 54 nt, synthetic construct
  misc_feature 1..54: note = V2-18-UTR
  source 1..54: mol_type = other RNA
gggaaataagagagaaaagaagaccccggcgtaagaagaaatataagagccacc

SEQ ID NO: 73 - RNA, 67 nt, synthetic construct
  misc_feature 1..67: note = CG1-UTR
  source 1..67: mol_type = other RNA
gggaaataagagagaaaagaagagtaagaagaaatataagagcgccccgcggcgccccgcggccacc

SEQ ID NO: 74 - RNA, 67 nt, synthetic construct
  misc_feature 1..67: note = CG1-1-UTR
  source 1..67: mol_type = other RNA
gggaaataagagagaaaagaagagtaagaagaaatataaggcgccccgcggcgccccgcgagccacc

SEQ ID NO: 75 - RNA, 67 nt, synthetic construct
  misc_feature 1..67: note = CG1-2-UTR
  source 1..67: mol_type = other RNA
gggaaataagagagaaaagaagagtaagaagaaatataagcgccccgcggcgccccgcggagccacc

SEQ ID NO: 76 - RNA, 67 nt, synthetic construct
  misc_feature 1..67: note = CG1-3-UTR
  source 1..67: mol_type = other RNA
gggaaataagagagaaaagaagagtaagaagaaatatagcgccccgcggcgccccgcgagagccacc

SEQ ID NO: 77 - RNA, 67 nt, synthetic construct
  misc_feature 1..67: note = CG1-4-UTR
  source 1..67: mol_type = other RNA
gggaaataagagagaaaagaagagtaagaagaaatatgcgccccgcggcgccccgcgaagagccacc

SEQ ID NO: 78 - RNA, 67 nt, synthetic construct
  misc_feature 1..67: note = CG1-5-UTR
  source 1..67: mol_type = other RNA
gggaaataagagagaaaagaagagtaagaagaaatagcgccccgcggcgccccgcgtaagagccacc

SEQ ID NO: 79 - RNA, 67 nt, synthetic construct
  misc_feature 1..67: note = CG1-6-UTR
  source 1..67: mol_type = other RNA
gggaaataagagagaaaagaagagtaagaagaaatgcgccccgcggcgccccgcgataagagccacc

SEQ ID NO: 80 - RNA, 67 nt, synthetic construct
  misc_feature 1..67: note = CG1-7-UTR
  source 1..67: mol_type = other RNA
gggaaataagagagaaaagaagagtaagaagaaagcgccccgcggcgccccgcgtataagagccacc

SEQ ID NO: 81 - RNA, 67 nt, synthetic construct
  misc_feature 1..67: note = CG1-8-UTR
  source 1..67: mol_type = other RNA
gggaaataagagagaaaagaagagtaagaagaagcgccccgcggcgccccgcgatataagagccacc

SEQ ID NO: 82 - RNA, 67 nt, synthetic construct
  misc_feature 1..67: note = CG1-9-UTR
  source 1..67: mol_type = other RNA
gggaaataagagagaaaagaagagtaagaagagcgccccgcggcgccccgcgaatataagagccacc

SEQ ID NO: 83 - RNA, 67 nt, synthetic construct
  misc_feature 1..67: note = CG1-10-UTR
  source 1..67: mol_type = other RNA
gggaaataagagagaaaagaagagtaagaaggcgccccgcggcgccccgcgaaatataagagccacc

SEQ ID NO: 84 - RNA, 67 nt, synthetic construct
  misc_feature 1..67: note = CG1-11-UTR
  source 1..67: mol_type = other RNA
gggaaataagagagaaaagaagagtaagaagcgccccgcggcgccccgcggaaatataagagccacc

SEQ ID NO: 85 - RNA, 67 nt, synthetic construct
  misc_feature 1..67: note = CG1-12-UTR
  source 1..67: mol_type = other RNA
gggaaataagagagaaaagaagagtaagagcgccccgcggcgccccgcgagaaatataagagccacc

SEQ ID NO: 86 - RNA, 67 nt, synthetic construct
  misc_feature 1..67: note = CG1-13-UTR
  source 1..67: mol_type = other RNA
gggaaataagagagaaaagaagagtaaggcgccccgcggcgccccgcgaagaaatataagagccacc

SEQ ID NO: 87 - RNA, 67 nt, synthetic construct
  misc_feature 1..67: note = CG1-14-UTR
  source 1..67: mol_type = other RNA
gggaaataagagagaaaagaagagtaagcgccccgcggcgccccgcggaagaaatataagagccacc

SEQ ID NO: 88 - RNA, 67 nt, synthetic construct
  misc_feature 1..67: note = CG1-15-UTR
  source 1..67: mol_type = other RNA
gggaaataagagagaaaagaagagtagcgccccgcggcgccccgcgagaagaaatataagagccacc

SEQ ID NO: 89 - RNA, 67 nt, synthetic construct
  misc_feature 1..67: note = CG1-16-UTR
  source 1..67: mol_type = other RNA
gggaaataagagagaaaagaagagtgcgccccgcggcgccccgcgaagaagaaatataagagccacc

SEQ ID NO: 90 - RNA, 67 nt, synthetic construct
  misc_feature 1..67: note = CG1-17-UTR
  source 1..67: mol_type = other RNA
gggaaataagagagaaaagaagaggcgccccgcggcgccccgcgtaagaagaaatataagagccacc

SEQ ID NO: 91 - RNA, 67 nt, synthetic construct
  misc_feature 1..67: note = CG1-18-UTR
  source 1..67: mol_type = other RNA
gggaaataagagagaaaagaagagcgccccgcggcgccccgcggtaagaagaaatataagagccacc

SEQ ID NO: 92 - RNA, 67 nt, synthetic construct
  misc_feature 1..67: note = CG2-UTR
  source 1..67: mol_type = other RNA
gggaaataagagagaaaagaagagtaagaagaaatataagacccgcccgccccgccccgccgccacc

SEQ ID NO: 93 - RNA, 67 nt, synthetic construct
  misc_feature 1..67: note = CG2-1-UTR
  source 1..67: mol_type = other RNA
gggaaataagagagaaaagaagagtaagaagaaatataagcccgcccgccccgccccgccagccacc

SEQ ID NO: 94 - RNA, 67 nt, synthetic construct
  misc_feature 1..67: note = CG2-2-UTR
  source 1..67: mol_type = other RNA
gggaaataagagagaaaagaagagtaagaagaaatataacccgcccgccccgccccgccgagccacc

SEQ ID NO: 95 - RNA, 67 nt, synthetic construct
  misc_feature 1..67: note = CG2-3-UTR
  source 1..67: mol_type = other RNA
gggaaataagagagaaaagaagagtaagaagaaatatacccgcccgccccgccccgccagagccacc

SEQ ID NO: 96 - RNA, 67 nt, synthetic construct
  misc_feature 1..67: note = CG2-4-UTR
  source 1..67: mol_type = other RNA
gggaaataagagagaaaagaagagtaagaagaaatatcccgcccgccccgccccgccaagagccacc

SEQ ID NO: 97 - RNA, 67 nt, synthetic construct
  misc_feature 1..67: note = CG2-5-UTR
  source 1..67: mol_type = other RNA
gggaaataagagagaaaagaagagtaagaagaaatacccgcccgccccgccccgcctaagagccacc

SEQ ID NO: 98 - RNA, 67 nt, synthetic construct
  misc_feature 1..67: note = CG2-6-UTR
  source 1..67: mol_type = other RNA
gggaaataagagagaaaagaagagtaagaagaaatcccgcccgccccgccccgccataagagccacc

SEQ ID NO: 99 - RNA, 67 nt, synthetic construct
  misc_feature 1..67: note = CG2-7-UTR
  source 1..67: mol_type = other RNA
gggaaataagagagaaaagaagagtaagaagaaacccgcccgccccgccccgcctataagagccacc

SEQ ID NO: 100 - RNA, 67 nt, synthetic construct
  misc_feature 1..67: note = CG2-8-UTR
  source 1..67: mol_type = other RNA
gggaaataagagagaaaagaagagtaagaagaacccgcccgccccgccccgccatataagagccacc

SEQ ID NO: 101 - RNA, 67 nt, synthetic construct
  misc_feature 1..67: note = CG2-9-UTR
  source 1..67: mol_type = other RNA
gggaaataagagagaaaagaagagtaagaagacccgcccgccccgccccgccaatataagagccacc

SEQ ID NO: 102 - RNA, 67 nt, synthetic construct
  misc_feature 1..67: note = CG2-10-UTR
  source 1..67: mol_type = other RNA
gggaaataagagagaaaagaagagtaagaagcccgcccgccccgccccgccaaatataagagccacc

SEQ ID NO: 103 - RNA, 67 nt, synthetic construct
  misc_feature 1..67: note = CG2-11-UTR
  source 1..67: mol_type = other RNA
gggaaataagagagaaaagaagagtaagaacccgcccgccccgccccgccgaaatataagagccacc

SEQ ID NO: 104 - RNA, 67 nt, synthetic construct
  misc_feature 1..67: note = CG2-12-UTR
  source 1..67: mol_type = other RNA
gggaaataagagagaaaagaagagtaagacccgcccgccccgccccgccagaaatataagagccacc

SEQ ID NO: 105 - RNA, 67 nt, synthetic construct
  misc_feature 1..67: note = CG2-13-UTR
  source 1..67: mol_type = other RNA
gggaaataagagagaaaagaagagtaagcccgcccgccccgccccgccaagaaatataagagccacc

SEQ ID NO: 106 - RNA, 67 nt, synthetic construct
  misc_feature 1..67: note = CG2-14-UTR
  source 1..67: mol_type = other RNA
gggaaataagagagaaaagaagagtaacccgcccgccccgccccgccgaagaaatataagagccacc

SEQ ID NO: 107 - RNA, 67 nt, synthetic construct
  misc_feature 1..67: note = CG2-15-UTR
  source 1..67: mol_type = other RNA
gggaaataagagagaaaagaagagtacccgcccgccccgccccgccagaagaaatataagagccacc

SEQ ID NO: 108 - RNA, 67 nt, synthetic construct
  misc_feature 1..67: note = CG2-16-UTR
  source 1..67: mol_type = other RNA
gggaaataagagagaaaagaagagtcccgcccgccccgccccgccaagaagaaatataagagccacc

SEQ ID NO: 109 - RNA, 67 nt, synthetic construct
  misc_feature 1..67: note = CG2-17-UTR
  source 1..67: mol_type = other RNA
gggaaataagagagaaaagaagagcccgcccgccccgccccgcctaagaagaaatataagagccacc

SEQ ID NO: 110 - RNA, 67 nt, synthetic construct
  misc_feature 1..67: note = CG2-18-UTR
  source 1..67: mol_type = other RNA
gggaaataagagagaaaagaagacccgcccgccccgccccgccgtaagaagaaatataagagccacc

SEQ ID NO: 111 - RNA, 53 nt, synthetic construct
  misc_feature 1..53: note = EK1-UTR
  source 1..53: mol_type = other RNA
gggaaataagagagaaaagaagagtaagaagaaatataagacccgccgccacc

SEQ ID NO: 112 - RNA, 53 nt, synthetic construct
  misc_feature 1..53: note = EK1-1-UTR
  source 1..53: mol_type = other RNA
gggaaataagagagaaaagaagagtaagaagaaatataagcccgccagccacc

SEQ ID NO: 113 - RNA, 53 nt, synthetic construct
  misc_feature 1..53: note = EK1-2-UTR
  source 1..53: mol_type = other RNA
gggaaataagagagaaaagaagagtaagaagaaatataacccgccgagccacc

SEQ ID NO: 114 - RNA, 53 nt, synthetic construct
  misc_feature 1..53: note = EK1-3-UTR
  source 1..53: mol_type = other RNA
gggaaataagagagaaaagaagagtaagaagaaatatacccgccagagccacc

SEQ ID NO: 115 - RNA, 53 nt, synthetic construct
  misc_feature 1..53: note = EK1-4-UTR
  source 1..53: mol_type = other RNA
gggaaataagagagaaaagaagagtaagaagaaatatcccgccaagagccacc

SEQ ID NO: 116 - RNA, 53 nt, synthetic construct
  misc_feature 1..53: note = EK1-5-UTR
  source 1..53: mol_type = other RNA
gggaaataagagagaaaagaagagtaagaagaaatacccgcctaagagccacc

SEQ ID NO: 117 - RNA, 53 nt, synthetic construct
  misc_feature 1..53: note = EK1-6-UTR
  source 1..53: mol_type = other RNA
gggaaataagagagaaaagaagagtaagaagaaatcccgccataagagccacc

SEQ ID NO: 118 - RNA, 53 nt, synthetic construct
  misc_feature 1..53: note = EK1-7-UTR
  source 1..53: mol_type = other RNA
gggaaataagagagaaaagaagagtaagaagaaacccgcctataagagccacc

SEQ ID NO: 119 - RNA, 53 nt, synthetic construct
  misc_feature 1..53: note = EK1-8-UTR
  source 1..53: mol_type = other RNA
gggaaataagagagaaaagaagagtaagaagaacccgccatataagagccacc

SEQ ID NO: 120 - RNA, 53 nt, synthetic construct
  misc_feature 1..53: note = EK1-9-UTR
  source 1..53: mol_type = other RNA
gggaaataagagagaaaagaagagtaagaagacccgccaatataagagccacc

SEQ ID NO: 121 - RNA, 53 nt, synthetic construct
  misc_feature 1..53: note = EK1-10-UTR
  source 1..53: mol_type = other RNA
gggaaataagagagaaaagaagagtaagaagcccgccaaatataagagccacc

SEQ ID NO: 122 - RNA, 53 nt, synthetic construct
  misc_feature 1..53: note = EK1-11-UTR
  source 1..53: mol_type = other RNA
gggaaataagagagaaaagaagagtaagaacccgccgaaatataagagccacc

SEQ ID NO: 123 - RNA, 53 nt, synthetic construct
  misc_feature 1..53: note = EK1-12-UTR
  source 1..53: mol_type = other RNA
gggaaataagagagaaaagaagagtaagacccgccagaaatataagagccacc

SEQ ID NO: 124 - RNA, 53 nt, synthetic construct
  misc_feature 1..53: note = EK1-13-UTR
  source 1..53: mol_type = other RNA
gggaaataagagagaaaagaagagtaagcccgccaagaaatataagagccacc

SEQ ID NO: 125 - RNA, 53 nt, synthetic construct
  misc_feature 1..53: note = EK1-14-UTR
  source 1..53: mol_type = other RNA
gggaaataagagagaaaagaagagtaacccgccgaagaaatataagagccacc

SEQ ID NO: 126 - RNA, 53 nt, synthetic construct
  misc_feature 1..53: note = EK1-15-UTR
  source 1..53: mol_type = other RNA
gggaaataagagagaaaagaagagtacccgccagaagaaatataagagccacc

SEQ ID NO: 127 - RNA, 53 nt, synthetic construct
  misc_feature 1..53: note = EK1-16-UTR
  source 1..53: mol_type = other RNA
gggaaataagagagaaaagaagagtcccgccaagaagaaatataagagccacc

SEQ ID NO: 128 - RNA, 53 nt, synthetic construct
  misc_feature 1..53: note = EK1-17-UTR
  source 1..53: mol_type = other RNA
gggaaataagagagaaaagaagagcccgcctaagaagaaatataagagccacc

SEQ ID NO: 129 - RNA, 53 nt, synthetic construct
  misc_feature 1..53: note = EK1-18-UTR
  source 1..53: mol_type = other RNA
gggaaataagagagaaaagaagacccgccgtaagaagaaatataagagccacc

SEQ ID NO: 130 - RNA, 53 nt, synthetic construct
  misc_feature 1..53: note = EK2-UTR
  source 1..53: mol_type = other RNA
gggaaataagagagaaaagaagagtaagaagaaatataagagccgccgccacc

SEQ ID NO: 131 - RNA, 53 nt, synthetic construct
  misc_feature 1..53: note = EK2-1-UTR
  source 1..53: mol_type = other RNA
gggaaataagagagaaaagaagagtaagaagaaatataaggccgccagccacc

SEQ ID NO: 132 - RNA, 53 nt, synthetic construct
  misc_feature 1..53: note = EK2-2-UTR
  source 1..53: mol_type = other RNA
gggaaataagagagaaaagaagagtaagaagaaatataagccgccgagccacc

SEQ ID NO: 133 - RNA, 53 nt, synthetic construct
  misc_feature 1..53: note = EK2-3-UTR
  source 1..53: mol_type = other RNA
gggaaataagagagaaaagaagagtaagaagaaatatagccgccagagccacc

SEQ ID NO: 134 - RNA, 53 nt, synthetic construct
  misc_feature 1..53: note = EK2-4-UTR
  source 1..53: mol_type = other RNA
gggaaataagagagaaaagaagagtaagaagaaatatgccgccaagagccacc

SEQ ID NO: 135 - RNA, 53 nt, synthetic construct
  misc_feature 1..53: note = EK2-5-UTR
  source 1..53: mol_type = other RNA
gggaaataagagagaaaagaagagtaagaagaaatagccgcctaagagccacc

SEQ ID NO: 136 - RNA, 53 nt, synthetic construct
  misc_feature 1..53: note = EK2-6-UTR
  source 1..53: mol_type = other RNA
gggaaataagagagaaaagaagagtaagaagaaatgccgccataagagccacc

SEQ ID NO: 137 - RNA, 53 nt, synthetic construct
  misc_feature 1..53: note = EK2-7-UTR
  source 1..53: mol_type = other RNA
gggaaataagagagaaaagaagagtaagaagaaagccgcctataagagccacc

SEQ ID NO: 138 - RNA, 53 nt, synthetic construct
  misc_feature 1..53: note = EK2-8-UTR
  source 1..53: mol_type = other RNA
gggaaataagagagaaaagaagagtaagaagaagccgccatataagagccacc

SEQ ID NO: 139 - RNA, 53 nt, synthetic construct
  misc_feature 1..53: note = EK2-9-UTR
  source 1..53: mol_type = other RNA
gggaaataagagagaaaagaagagtaagaagagccgccaatataagagccacc

SEQ ID NO: 140 - RNA, 53 nt, synthetic construct
  misc_feature 1..53: note = EK2-10-UTR
  source 1..53: mol_type = other RNA
gggaaataagagagaaaagaagagtaagaaggccgccaaatataagagccacc

SEQ ID NO: 141 - RNA, 53 nt, synthetic construct
  misc_feature 1..53: note = EK2-11-UTR
  source 1..53: mol_type = other RNA
gggaaataagagagaaaagaagagtaagaagccgccgaaatataagagccacc

SEQ ID NO: 142 - RNA, 53 nt, synthetic construct
  misc_feature 1..53: note = EK2-12-UTR
  source 1..53: mol_type = other RNA
gggaaataagagagaaaagaagagtaagagccgccagaaatataagagccacc

SEQ ID NO: 143 - RNA, 53 nt, synthetic construct
  misc_feature 1..53: note = EK2-13-UTR
  source 1..53: mol_type = other RNA
gggaaataagagagaaaagaagagtaaggccgccaagaaatataagagccacc

SEQ ID NO: 144 - RNA, 53 nt, synthetic construct
  misc_feature 1..53: note = EK2-14-UTR
  source 1..53: mol_type = other RNA
gggaaataagagagaaaagaagagtaagccgccgaagaaatataagagccacc

SEQ ID NO: 145 - RNA, 53 nt, synthetic construct
  misc_feature 1..53: note = EK2-15-UTR
  source 1..53: mol_type = other RNA
gggaaataagagagaaaagaagagtagccgccagaagaaatataagagccacc

SEQ ID NO: 146 - RNA, 53 nt, synthetic construct
  misc_feature 1..53: note = EK2-16-UTR
  source 1..53: mol_type = other RNA
gggaaataagagagaaaagaagagtgccgccaagaagaaatataagagccacc

SEQ ID NO: 147 - RNA, 53 nt, synthetic construct
  misc_feature 1..53: note = EK2-17-UTR
  source 1..53: mol_type = other RNA
gggaaataagagagaaaagaagaggccgcctaagaagaaatataagagccacc

SEQ ID NO: 148 - RNA, 53 nt, synthetic construct
  misc_feature 1..53: note = EK2-18-UTR
  source 1..53: mol_type = other RNA
gggaaataagagagaaaagaagagccgccgtaagaagaaatataagagccacc

SEQ ID NO: 149 - RNA, 53 nt, synthetic construct
  misc_feature 1..53: note = EK3-UTR
  source 1..53: mol_type = other RNA
gggaaataagagagaaaagaagagtaagaagaaatataagaccgccggccacc

SEQ ID NO: 150 - RNA, 53 nt, synthetic construct; identical to SEQ ID NO: 132
  misc_feature 1..53: note = EK3-1-UTR
  source 1..53: mol_type = other RNA

SEQ ID NO: 151 - RNA, 53 nt, synthetic construct
  misc_feature 1..53: note = EK3-2-UTR
  source 1..53: mol_type = other RNA
gggaaataagagagaaaagaagagtaagaagaaatataaccgccggagccacc

SEQ ID NO: 152 - RNA, 53 nt, synthetic construct
  misc_feature 1..53: note = EK3-3-UTR
  source 1..53: mol_type = other RNA
gggaaataagagagaaaagaagagtaagaagaaatataccgccgagagccacc

SEQ ID NO: 153 - RNA, 53 nt, synthetic construct
  misc_feature 1..53: note = EK3-4-UTR
  source 1..53: mol_type = other RNA
gggaaataagagagaaaagaagagtaagaagaaatatccgccgaagagccacc

SEQ ID NO: 154 - RNA, 53 nt, synthetic construct
  misc_feature 1..53: note = EK3-5-UTR
  source 1..53: mol_type = other RNA
gggaaataagagagaaaagaagagtaagaagaaataccgccgtaagagccacc

SEQ ID NO: 155 - RNA, 53 nt, synthetic construct
  misc_feature 1..53: note = EK3-6-UTR
  source 1..53: mol_type = other RNA
gggaaataagagagaaaagaagagtaagaagaaatccgccgataagagccacc

SEQ ID NO: 156 - RNA, 53 nt, synthetic construct
  misc_feature 1..53: note = EK3-7-UTR
  source 1..53: mol_type = other RNA
gggaaataagagagaaaagaagagtaagaagaaaccgccgtataagagccacc

SEQ ID NO: 157 - RNA, 53 nt, synthetic construct
  misc_feature 1..53: note = EK3-8-UTR
  source 1..53: mol_type = other RNA
gggaaataagagagaaaagaagagtaagaagaaccgccgatataagagccacc

SEQ ID NO: 158 - RNA, 53 nt, synthetic construct
  misc_feature 1..53: note = EK3-9-UTR
  source 1..53: mol_type = other RNA
gggaaataagagagaaaagaagagtaagaagaccgccgaatataagagccacc

SEQ ID NO: 159 - RNA, 53 nt, synthetic construct; identical to SEQ ID NO: 141
  misc_feature 1..53: note = EK3-10-UTR
  source 1..53: mol_type = other RNA

SEQ ID NO: 160 - RNA, 53 nt, synthetic construct
  misc_feature 1..53: note = EK3-11-UTR
  source 1..53: mol_type = other RNA
gggaaataagagagaaaagaagagtaagaaccgccggaaatataagagccacc

SEQ ID NO: 161 - RNA, 53 nt, synthetic construct
  misc_feature 1..53: note = EK3-12-UTR
  source 1..53: mol_type = other RNA
gggaaataagagagaaaagaagagtaagaccgccgagaaatataagagccacc

SEQ ID NO: 162 - RNA, 53 nt, synthetic construct; identical to SEQ ID NO: 144
  misc_feature 1..53: note = EK3-13-UTR
  source 1..53: mol_type = other RNA

SEQ ID NO: 163 - RNA, 53 nt, synthetic construct
  misc_feature 1..53: note = EK3-14-UTR
  source 1..53: mol_type = other RNA
gggaaataagagagaaaagaagagtaaccgccggaagaaatataagagccacc

SEQ ID NO: 164 - RNA, 53 nt, synthetic construct
  misc_feature 1..53: note = EK3-15-UTR
  source 1..53: mol_type = other RNA
gggaaataagagagaaaagaagagtaccgccgagaagaaatataagagccacc

SEQ ID NO: 165 - RNA, 53 nt, synthetic construct
  misc_feature 1..53: note = EK3-16-UTR
  source 1..53: mol_type = other RNA
gggaaataagagagaaaagaagagtccgccgaagaagaaatataagagccacc

SEQ ID NO: 166 - RNA, 53 nt, synthetic construct; identical to SEQ ID NO: 148
  misc_feature 1..53: note = EK3-17-UTR
  source 1..53: mol_type = other RNA

SEQ ID NO: 167 - RNA, 53 nt, synthetic construct
  misc_feature 1..53: note = EK3-18-UTR
  source 1..53: mol_type = other RNA
gggaaataagagagaaaagaagaccgccggtaagaagaaatataagagccacc

SEQ ID NO: 168 - RNA, 56 nt, synthetic construct
  misc_feature 1..56: note = (CCG)3-UTR
  source 1..56: mol_type = other RNA
gggaaataagagagaaaagaagagtaagaagaaatataagaccgccgccggccacc

SEQ ID NO: 169 - RNA, 56 nt, synthetic construct
  misc_feature 1..56: note = (CCG)3-1-UTR
  source 1..56: mol_type = other RNA
gggaaataagagagaaaagaagagtaagaagaaatataagccgccgccgagccacc

SEQ ID NO: 170 - RNA, 56 nt, synthetic construct
  misc_feature 1..56: note = (CCG)3-2-UTR
  source 1..56: mol_type = other RNA
gggaaataagagagaaaagaagagtaagaagaaatataaccgccgccggagccacc

SEQ ID NO: 171 - RNA, 56 nt, synthetic construct
  misc_feature 1..56: note = (CCG)3-3-UTR
  source 1..56: mol_type = other RNA
gggaaataagagagaaaagaagagtaagaagaaatataccgccgccgagagccacc

SEQ ID NO: 172 - RNA, 56 nt, synthetic construct
  misc_feature 1..56: note = (CCG)3-4-UTR
  source 1..56: mol_type = other RNA
gggaaataagagagaaaagaagagtaagaagaaatatccgccgccgaagagccacc

SEQ ID NO: 173 - RNA, 56 nt, synthetic construct
  misc_feature 1..56: note = (CCG)3-5-UTR
  source 1..56: mol_type = other RNA
gggaaataagagagaaaagaagagtaagaagaaataccgccgccgtaagagccacc

SEQ ID NO: 174 - RNA, 56 nt, synthetic construct
  misc_feature 1..56: note = (CCG)3-6-UTR
  source 1..56: mol_type = other RNA
gggaaataagagagaaaagaagagtaagaagaaatccgccgccgataagagccacc

SEQ ID NO: 175 - RNA, 56 nt, synthetic construct
  misc_feature 1..56: note = (CCG)3-7-UTR
  source 1..56: mol_type = other RNA
gggaaataagagagaaaagaagagtaagaagaaaccgccgccgtataagagccacc

SEQ ID NO: 176 - RNA, 56 nt, synthetic construct
  misc_feature 1..56: note = (CCG)3-8-UTR
  source 1..56: mol_type = other RNA
gggaaataagagagaaaagaagagtaagaagaaccgccgccgatataagagccacc

SEQ ID NO: 177 - RNA, 56 nt, synthetic construct
  misc_feature 1..56: note = (CCG)3-9-UTR
  source 1..56: mol_type = other RNA
gggaaataagagagaaaagaagagtaagaagaccgccgccgaatataagagccacc

SEQ ID NO: 178 - RNA, 56 nt, synthetic construct
  misc_feature 1..56: note = (CCG)3-10-UTR
  source 1..56: mol_type = other RNA
gggaaataagagagaaaagaagagtaagaagccgccgccgaaatataagagccacc

SEQ ID NO: 179 - RNA, 56 nt, synthetic construct
  misc_feature 1..56: note = (CCG)3-11-UTR
  source 1..56: mol_type = other RNA
gggaaataagagagaaaagaagagtaagaaccgccgccggaaatataagagccacc

SEQ ID NO: 180 - RNA, 56 nt, synthetic construct
  misc_feature 1..56: note = (CCG)3-12-UTR
  source 1..56: mol_type = other RNA
gggaaataagagagaaaagaagagtaagaccgccgccgagaaatataagagccacc

SEQ ID NO: 181 - RNA, 56 nt, synthetic construct
  misc_feature 1..56: note = (CCG)3-13-UTR
  source 1..56: mol_type = other RNA
gggaaataagagagaaaagaagagtaagccgccgccgaagaaatataagagccacc

SEQ ID NO: 182 - RNA, 56 nt, synthetic construct
  misc_feature 1..56: note = (CCG)3-14-UTR
  source 1..56: mol_type = other RNA
gggaaataagagagaaaagaagagtaaccgccgccggaagaaatataagagccacc

SEQ ID NO: 183 - RNA, 56 nt, synthetic construct
  misc_feature 1..56: note = (CCG)3-15-UTR
  source 1..56: mol_type = other RNA
gggaaataagagagaaaagaagagtaccgccgccgagaagaaatataagagccacc

SEQ ID NO: 184 - RNA, 56 nt, synthetic construct
  misc_feature 1..56: note = (CCG)3-16-UTR
  source 1..56: mol_type = other RNA
gggaaataagagagaaaagaagagtccgccgccgaagaagaaatataagagccacc

SEQ ID NO: 185 - RNA, 56 nt, synthetic construct
  misc_feature 1..56: note = (CCG)3-17-UTR
  source 1..56: mol_type = other RNA
gggaaataagagagaaaagaagagccgccgccgtaagaagaaatataagagccacc

SEQ ID NO: 186 - RNA, 56 nt, synthetic construct
  misc_feature 1..56: note = (CCG)3-18-UTR
  source 1..56: mol_type = other RNA
gggaaataagagagaaaagaagaccgccgccggtaagaagaaatataagagccacc

SEQ ID NO: 187 - RNA, 59 nt, synthetic construct
  misc_feature 1..59: note = (CCG)4-UTR
  source 1..59: mol_type = other RNA
gggaaataagagagaaaagaagagtaagaagaaatataagaccgccgccgccggccacc

SEQ ID NO: 188 - RNA, 59 nt, synthetic construct
  misc_feature 1..59: note = (CCG)4-1-UTR
  source 1..59: mol_type = other RNA
gggaaataagagagaaaagaagagtaagaagaaatataagccgccgccgccgagccacc

SEQ ID NO: 189 - RNA, 59 nt, synthetic construct
  misc_feature 1..59: note = (CCG)4-2-UTR
  source 1..59: mol_type = other RNA
gggaaataagagagaaaagaagagtaagaagaaatataaccgccgccgccggagccacc

SEQ ID NO: 190 - RNA, 59 nt, synthetic construct
  misc_feature 1..59: note = (CCG)4-3-UTR
  source 1..59: mol_type = other RNA
gggaaataagagagaaaagaagagtaagaagaaatataccgccgccgccgagagccacc

SEQ ID NO: 191 - RNA, 59 nt, synthetic construct
  misc_feature 1..59: note = (CCG)4-4-UTR
  source 1..59: mol_type = other RNA
gggaaataagagagaaaagaagagtaagaagaaatatccgccgccgccgaagagccacc

SEQ ID NO: 192 - RNA, 59 nt, synthetic construct
  misc_feature 1..59: note = (CCG)4-5-UTR
  source 1..59: mol_type = other RNA
gggaaataagagagaaaagaagagtaagaagaaataccgccgccgccgtaagagccacc

SEQ ID NO: 193 - RNA, 59 nt, synthetic construct
  misc_feature 1..59: note = (CCG)4-6-UTR
  source 1..59: mol_type = other RNA
gggaaataagagagaaaagaagagtaagaagaaatccgccgccgccgataagagccacc

SEQ ID NO: 194 - RNA, 59 nt, synthetic construct
  misc_feature 1..59: note = (CCG)4-7-UTR
  source 1..59: mol_type = other RNA
gggaaataagagagaaaagaagagtaagaagaaaccgccgccgccgtataagagccacc

SEQ ID NO: 195 - RNA, 59 nt, synthetic construct
  misc_feature 1..59: note = (CCG)4-8-UTR
  source 1..59: mol_type = other RNA
gggaaataagagagaaaagaagagtaagaagaaccgccgccgccgatataagagccacc

SEQ ID NO: 196 - RNA, 59 nt, synthetic construct
  misc_feature 1..59: note = (CCG)4-9-UTR
  source 1..59: mol_type = other RNA
gggaaataagagagaaaagaagagtaagaagaccgccgccgccgaatataagagccacc

SEQ ID NO: 197 - RNA, 59 nt, synthetic construct
  misc_feature 1..59: note = (CCG)4-10-UTR
  source 1..59: mol_type = other RNA
gggaaataagagagaaaagaagagtaagaagccgccgccgccgaaatataagagccacc

SEQ ID NO: 198 - RNA, 59 nt, synthetic construct
  misc_feature 1..59: note = (CCG)4-11-UTR
  source 1..59: mol_type = other RNA
gggaaataagagagaaaagaagagtaagaaccgccgccgccggaaatataagagccacc

SEQ ID NO: 199 - RNA, 59 nt, synthetic construct
  misc_feature 1..59: note = (CCG)4-12-UTR
  source 1..59: mol_type = other RNA
gggaaataagagagaaaagaagagtaagaccgccgccgccgagaaatataagagccacc

SEQ ID NO: 200 - RNA, 59 nt, synthetic construct
  misc_feature 1..59: note = (CCG)4-13-UTR
  source 1..59: mol_type = other RNA
gggaaataagagagaaaagaagagtaagccgccgccgccgaagaaatataagagccacc

SEQ ID NO: 201 - RNA, 59 nt, synthetic construct
  misc_feature 1..59: note = (CCG)4-14-UTR
  source 1..59: mol_type = other RNA
gggaaataagagagaaaagaagagtaaccgccgccgccggaagaaatataagagccacc

SEQ ID NO: 202 - RNA, 59 nt, synthetic construct
  misc_feature 1..59: note = (CCG)4-15-UTR
  source 1..59: mol_type = other RNA
gggaaataagagagaaaagaagagtaccgccgccgccgagaagaaatataagagccacc

SEQ ID NO: 203 - RNA, 59 nt, synthetic construct
  misc_feature 1..59: note = (CCG)4-16-UTR
  source 1..59: mol_type = other RNA
gggaaataagagagaaaagaagagtccgccgccgccgaagaagaaatataagagccacc

SEQ ID NO: 204 - RNA, 59 nt, synthetic construct
  misc_feature 1..59: note = (CCG)4-17-UTR
  source 1..59: mol_type = other RNA
gggaaataagagagaaaagaagagccgccgccgccgtaagaagaaatataagagccacc

SEQ ID NO: 205 - RNA, 59 nt, synthetic construct
  misc_feature 1..59: note = (CCG)4-18-UTR
  source 1..59: mol_type = other RNA
gggaaataagagagaaaagaagaccgccgccgccggtaagaagaaatataagagccacc

SEQ ID NO: 206 - RNA, 62 nt, synthetic construct
  misc_feature 1..62: note = (CCG)5-UTR
  source 1..62: mol_type = other RNA
gggaaataagagagaaaagaagagtaagaagaaatataagaccgccgccgccgccggccacc

SEQ ID NO: 207 - RNA, 62 nt, synthetic construct
  misc_feature 1..62: note = (CCG)5-1-UTR
  source 1..62: mol_type = other RNA
gggaaataagagagaaaagaagagtaagaagaaatataagccgccgccgccgccgagccacc

SEQ ID NO: 208 - RNA, 62 nt, synthetic construct
  misc_feature 1..62: note = (CCG)5-2-UTR
  source 1..62: mol_type = other RNA
gggaaataagagagaaaagaagagtaagaagaaatataaccgccgccgccgccggagccacc

SEQ ID NO: 209 - RNA, 62 nt, synthetic construct
  misc_feature 1..62: note = (CCG)5-3-UTR
  source 1..62: mol_type = other RNA
gggaaataagagagaaaagaagagtaagaagaaatataccgccgccgccgccgagagccacc

SEQ ID NO: 210 - RNA, 62 nt, synthetic construct
  misc_feature 1..62: note = (CCG)5-4-UTR
  source 1..62: mol_type = other RNA
gggaaataagagagaaaagaagagtaagaagaaatatccgccgccgccgccgaagagccacc

SEQ ID NO: 211 - RNA, 62 nt, synthetic construct
  misc_feature 1..62: note = (CCG)5-5-UTR
  source 1..62: mol_type = other RNA
gggaaataagagagaaaagaagagtaagaagaaataccgccgccgccgccgtaagagccacc

SEQ ID NO: 212 - RNA, 62 nt, synthetic construct
  misc_feature 1..62: note = (CCG)5-6-UTR
  source 1..62: mol_type = other RNA
gggaaataagagagaaaagaagagtaagaagaaatccgccgccgccgccgataagagccacc

SEQ ID NO: 213 - RNA, 62 nt, synthetic construct
  misc_feature 1..62: note = (CCG)5-7-UTR
  source 1..62: mol_type = other RNA
gggaaataagagagaaaagaagagtaagaagaaaccgccgccgccgccgtataagagccacc

SEQ ID NO: 214 - RNA, 62 nt, synthetic construct
  misc_feature 1..62: note = (CCG)5-8-UTR
  source 1..62: mol_type = other RNA
gggaaataagagagaaaagaagagtaagaagaaccgccgccgccgccgatataagagccacc

SEQ ID NO: 215 - RNA, 62 nt, synthetic construct
  misc_feature 1..62: note = (CCG)5-9-UTR
  source 1..62: mol_type = other RNA
gggaaataagagagaaaagaagagtaagaagaccgccgccgccgccgaatataagagccacc

SEQ ID NO: 216 - RNA, 62 nt, synthetic construct
  misc_feature 1..62: note = (CCG)5-10-UTR
  source 1..62: mol_type = other RNA
gggaaataagagagaaaagaagagtaagaagccgccgccgccgccgaaatataagagccacc

SEQ ID NO: 217 - RNA, 62 nt, synthetic construct
  misc_feature 1..62: note = (CCG)5-11-UTR
  source 1..62: mol_type = other RNA
gggaaataagagagaaaagaagagtaagaaccgccgccgccgccggaaatataagagccacc

SEQ ID NO: 218 - RNA, 62 nt, synthetic construct
  misc_feature 1..62: note = (CCG)5-12-UTR
  source 1..62: mol_type = other RNA
gggaaataagagagaaaagaagagtaagaccgccgccgccgccgagaaatataagagccacc

SEQ ID NO: 219 - RNA, 62 nt, synthetic construct
  misc_feature 1..62: note = (CCG)5-13-UTR
  source 1..62: mol_type = other RNA
gggaaataagagagaaaagaagagtaagccgccgccgccgccgaagaaatataagagccacc

SEQ ID NO: 220 - RNA, 62 nt, synthetic construct
  misc_feature 1..62: note = (CCG)5-14-UTR
  source 1..62: mol_type = other RNA
gggaaataagagagaaaagaagagtaaccgccgccgccgccggaagaaatataagagccacc

SEQ ID NO: 221 - RNA, 62 nt, synthetic construct
  misc_feature 1..62: note = (CCG)5-15-UTR
  source 1..62: mol_type = other RNA
gggaaataagagagaaaagaagagtaccgccgccgccgccgagaagaaatataagagccacc

SEQ ID NO: 222 - RNA, 62 nt, synthetic construct
  misc_feature 1..62: note = (CCG)5-16-UTR
  source 1..62: mol_type = other RNA
gggaaataagagagaaaagaagagtccgccgccgccgccgaagaagaaatataagagccacc

SEQ ID NO: 223 - RNA, 62 nt, synthetic construct
  misc_feature 1..62: note = (CCG)5-17-UTR
  source 1..62: mol_type = other RNA
gggaaataagagagaaaagaagagccgccgccgccgccgtaagaagaaatataagagccacc

SEQ ID NO: 224 - RNA, 62 nt, synthetic construct
  misc_feature 1..62: note = (CCG)5-18-UTR
  source 1..62: mol_type = other RNA
gggaaataagagagaaaagaagaccgccgccgccgccggtaagaagaaatataagagccacc

SEQ ID NO: 225 - RNA, 65 nt, synthetic construct
  misc_feature 1..65: note = (CCG)6-UTR
  source 1..65: mol_type = other RNA
gggaaataagagagaaaagaagagtaagaagaaatataagaccgccgccgccgccgccggccacc

SEQ ID NO: 226 - RNA, 65 nt, synthetic construct
  misc_feature 1..65: note = (CCG)6-1-UTR
  source 1..65: mol_type = other RNA
gggaaataagagagaaaagaagagtaagaagaaatataagccgccgccgccgccgccgagccacc

SEQ ID NO: 227 - RNA, 65 nt, synthetic construct
  misc_feature 1..65: note = (CCG)6-2-UTR
  source 1..65: mol_type = other RNA
gggaaataagagagaaaagaagagtaagaagaaatataaccgccgccgccgccgccggagccacc

SEQ ID NO: 228 - RNA, 65 nt, synthetic construct
  misc_feature 1..65: note = (CCG)6-3-UTR
  source 1..65: mol_type = other RNA
gggaaataagagagaaaagaagagtaagaagaaatataccgccgccgccgccgccgagagccacc

SEQ ID NO: 229 - RNA, 65 nt, synthetic construct
  misc_feature 1..65: note = (CCG)6-4-UTR
  source 1..65: mol_type = other RNA
gggaaataagagagaaaagaagagtaagaagaaatatccgccgccgccgccgccgaagagccacc

SEQ ID NO: 230 - RNA, 65 nt, synthetic construct
  misc_feature 1..65: note = (CCG)6-5-UTR
  source 1..65: mol_type = other RNA
gggaaataagagagaaaagaagagtaagaagaaataccgccgccgccgccgccgtaagagccacc

SEQ ID NO: 231 - RNA, 65 nt, synthetic construct
  misc_feature 1..65: note = (CCG)6-6-UTR
  source 1..65: mol_type = other RNA
gggaaataagagagaaaagaagagtaagaagaaatccgccgccgccgccgccgataagagccacc

SEQ ID NO: 232 - RNA, 65 nt, synthetic construct
  misc_feature 1..65: note = (CCG)6-7-UTR
  source 1..65: mol_type = other RNA
gggaaataagagagaaaagaagagtaagaagaaaccgccgccgccgccgccgtataagagccacc

SEQ ID NO: 233 - RNA, 65 nt, synthetic construct
  misc_feature 1..65: note = (CCG)6-8-UTR
  source 1..65: mol_type = other RNA
gggaaataagagagaaaagaagagtaagaagaaccgccgccgccgccgccgatataagagccacc

SEQ ID NO: 234 - RNA, 65 nt, synthetic construct
  misc_feature 1..65: note = (CCG)6-9-UTR
  source 1..65: mol_type = other RNA
gggaaataagagagaaaagaagagtaagaagaccgccgccgccgccgccgaatataagagccacc

SEQ ID NO: 235 - RNA, 65 nt, synthetic construct
  misc_feature 1..65: note = (CCG)6-10-UTR
  source 1..65: mol_type = other RNA
gggaaataagagagaaaagaagagtaagaagccgccgccgccgccgccgaaatataagagccacc

SEQ ID NO: 236 - RNA, 65 nt, synthetic construct
  misc_feature 1..65: note = (CCG)6-11-UTR
  source 1..65: mol_type = other RNA
gggaaataagagagaaaagaagagtaagaaccgccgccgccgccgccggaaatataagagccacc

SEQ ID NO: 237 - RNA, 65 nt, synthetic construct
  misc_feature 1..65: note = (CCG)6-12-UTR
  source 1..65: mol_type = other RNA
gggaaataagagagaaaagaagagtaagaccgccgccgccgccgccgagaaatataagagccacc

SEQ ID NO: 238 - RNA, 65 nt, synthetic construct
  misc_feature 1..65: note = (CCG)6-13-UTR
  source 1..65: mol_type = other RNA
gggaaataagagagaaaagaagagtaagccgccgccgccgccgccgaagaaatataagagccacc

SEQ ID NO: 239 - RNA, 65 nt, synthetic construct
  misc_feature 1..65: note = (CCG)6-14-UTR
  source 1..65: mol_type = other RNA
gggaaataagagagaaaagaagagtaaccgccgccgccgccgccggaagaaatataagagccacc

SEQ ID NO: 240 - RNA, 65 nt, synthetic construct
  misc_feature 1..65: note = (CCG)6-15-UTR
  source 1..65: mol_type = other RNA
gggaaataagagagaaaagaagagtaccgccgccgccgccgccgagaagaaatataagagccacc

SEQ ID NO: 241 - RNA, 65 nt, synthetic construct
  misc_feature 1..65: note = (CCG)6-16-UTR
  source 1..65: mol_type = other RNA
gggaaataagagagaaaagaagagtccgccgccgccgccgccgaagaagaaatataagagccacc

SEQ ID NO: 242 - RNA, 65 nt, synthetic construct
  misc_feature 1..65: note = (CCG)6-17-UTR
  source 1..65: mol_type = other RNA
gggaaataagagagaaaagaagagccgccgccgccgccgccgtaagaagaaatataagagccacc

SEQ ID NO: 243 - RNA, 65 nt, synthetic construct
  misc_feature 1..65: note = (CCG)6-18-UTR
  source 1..65: mol_type = other RNA
gggaaataagagagaaaagaagaccgccgccgccgccgccggtaagaagaaatataagagccacc

SEQ ID NO: 244 - RNA, 68 nt, synthetic construct
  misc_feature 1..68: note = (CCG)7-UTR
  source 1..68: mol_type = other RNA
gggaaataagagagaaaagaagagtaagaagaaatataagaccgccgccgccgccgccgccggccacc

SEQ ID NO: 245 - RNA, 68 nt, synthetic construct
  misc_feature 1..68: note = (CCG)7-1-UTR
  source 1..68: mol_type = other RNA
gggaaataagagagaaaagaagagtaagaagaaatataagccgccgccgccgccgccgccgagccacc

SEQ ID NO: 246 - RNA, 68 nt, synthetic construct
  misc_feature 1..68: note = (CCG)7-2-UTR
  source 1..68: mol_type = other RNA
gggaaataagagagaaaagaagagtaagaagaaatataaccgccgccgccgccgccgccggagccacc

SEQ ID NO: 247 - RNA, 68 nt, synthetic construct
  misc_feature 1..68: note = (CCG)7-3-UTR
  source 1..68: mol_type = other RNA
gggaaataagagagaaaagaagagtaagaagaaatataccgccgccgccgccgccgccgagagccacc

SEQ ID NO: 248 - RNA, 68 nt, synthetic construct
  misc_feature 1..68: note = (CCG)7-4-UTR
  source 1..68: mol_type = other RNA
gggaaataagagagaaaagaagagtaagaagaaatatccgccgccgccgccgccgccgaagagccacc

SEQ ID NO: 249 - RNA, 68 nt, synthetic construct
  misc_feature 1..68: note = (CCG)7-5-UTR
  source 1..68: mol_type = other RNA
gggaaataagagagaaaagaagagtaagaagaaataccgccgccgccgccgccgccgtaagagccacc

SEQ ID NO: 250 - RNA, 68 nt, synthetic construct
  misc_feature 1..68: note = (CCG)7-6-UTR
  source 1..68: mol_type = other RNA
gggaaataagagagaaaagaagagtaagaagaaatccgccgccgccgccgccgccgataagagccacc

SEQ ID NO: 251 - RNA, 68 nt, synthetic construct
  misc_feature 1..68: note = (CCG)7-7-UTR
  source 1..68: mol_type = other RNA
gggaaataagagagaaaagaagagtaagaagaaaccgccgccgccgccgccgccgtataagagccacc

SEQ ID NO: 252 - RNA, 68 nt, synthetic construct
  misc_feature 1..68: note = (CCG)7-8-UTR
  source 1..68: mol_type = other RNA
gggaaataagagagaaaagaagagtaagaagaaccgccgccgccgccgccgccgatataagagccacc

SEQ ID NO: 253 - RNA, 68 nt, synthetic construct
  misc_feature 1..68: note = (CCG)7-9-UTR
  source 1..68: mol_type = other RNA
gggaaataagagagaaaagaagagtaagaagaccgccgccgccgccgccgccgaatataagagccacc

SEQ ID NO: 254 - RNA, 68 nt, synthetic construct
  misc_feature 1..68: note = (CCG)7-10-UTR
  source 1..68: mol_type = other RNA
gggaaataagagagaaaagaagagtaagaagccgccgccgccgccgccgccgaaatataagagccacc

SEQ ID NO: 255 - RNA, 68 nt, synthetic construct
  misc_feature 1..68: note = (CCG)7-11-UTR
  source 1..68: mol_type = other RNA
gggaaataagagagaaaagaagagtaagaaccgccgccgccgccgccgccggaaatataagagccacc

SEQ ID NO: 256 - RNA, 68 nt, synthetic construct
  misc_feature 1..68: note = (CCG)7-12-UTR
  source 1..68: mol_type = other RNA
gggaaataagagagaaaagaagagtaagaccgccgccgccgccgccgccgagaaatataagagccacc

SEQ ID NO: 257 - RNA, 68 nt, synthetic construct
  misc_feature 1..68: note = (CCG)7-13-UTR
  source 1..68: mol_type = other RNA
gggaaataagagagaaaagaagagtaagccgccgccgccgccgccgccgaagaaatataagagccacc

SEQ ID NO: 258 - RNA, 68 nt, synthetic construct
  misc_feature 1..68: note = (CCG)7-14-UTR
  source 1..68: mol_type = other RNA
gggaaataagagagaaaagaagagtaaccgccgccgccgccgccgccggaagaaatataagagccacc

SEQ ID NO: 259 - RNA, 68 nt, synthetic construct
  misc_feature 1..68: note = (CCG)7-15-UTR
  source 1..68: mol_type = other RNA
gggaaataagagagaaaagaagagtaccgccgccgccgccgccgccgagaagaaatataagagccacc

SEQ ID NO: 260 - RNA, 68 nt, synthetic construct
  misc_feature 1..68: note = (CCG)7-16-UTR
  source 1..68: mol_type = other RNA
gggaaataagagagaaaagaagagtccgccgccgccgccgccgccgaagaagaaatataagagccacc

SEQ ID NO: 261 - RNA, 68 nt, synthetic construct
  misc_feature 1..68: note = (CCG)7-17-UTR
  source 1..68: mol_type = other RNA
gggaaataagagagaaaagaagagccgccgccgccgccgccgccgtaagaagaaatataagagccacc

SEQ ID NO: 262 - RNA, 68 nt, synthetic construct
  misc_feature 1..68: note = (CCG)7-18-UTR
  source 1..68: mol_type = other RNA
gggaaataagagagaaaagaagaccgccgccgccgccgccgccggtaagaagaaatataagagccacc

SEQ ID NO: 263 - RNA, 71 nt, synthetic construct
  misc_feature 1..71: note = (CCG)8-UTR
  source 1..71: mol_type = other RNA
gggaaataagagagaaaagaagagtaagaagaaatataagaccgccgccgccgccgccgccgccggccacc

SEQ ID NO: 264 - RNA, 71 nt, synthetic construct
  misc_feature 1..71: note = (CCG)8-1-UTR
  source 1..71: mol_type = other RNA
gggaaataagagagaaaagaagagtaagaagaaatataagccgccgccgccgccgccgccgccgagccacc

SEQ ID NO: 265 - RNA, 71 nt, synthetic construct
  misc_feature 1..71: note = (CCG)8-2-UTR
  source 1..71: mol_type = other RNA
gggaaataagagagaaaagaagagtaagaagaaatataaccgccgccgccgccgccgccgccggagccacc

SEQ ID NO: 266 - RNA, 71 nt, synthetic construct
  misc_feature 1..71: note = (CCG)8-3-UTR
  source 1..71: mol_type = other RNA
gggaaataagagagaaaagaagagtaagaagaaatataccgccgccgccgccgccgccgccgagagccacc

SEQ ID NO: 267 - RNA, 71 nt, synthetic construct
  misc_feature 1..71: note = (CCG)8-4-UTR
  source 1..71: mol_type = other RNA
gggaaataagagagaaaagaagagtaagaagaaatatccgccgccgccgccgccgccgccgaagagccacc

SEQ ID NO: 268 - RNA, 71 nt, synthetic construct
  misc_feature 1..71: note = (CCG)8-5-UTR
  source 1..71: mol_type = other RNA
gggaaataagagagaaaagaagagtaagaagaaataccgccgccgccgccgccgccgccgtaagagccacc

SEQ ID NO: 269 - RNA, 71 nt, synthetic construct
  misc_feature 1..71: note = (CCG)8-6-UTR
  source 1..71: mol_type = other RNA
gggaaataagagagaaaagaagagtaagaagaaatccgccgccgccgccgccgccgccgataagagccacc

SEQ ID NO: 270 - RNA, 71 nt, synthetic construct
  misc_feature 1..71: note = (CCG)8-7-UTR
  source 1..71: mol_type = other RNA
gggaaataagagagaaaagaagagtaagaagaaaccgccgccgccgccgccgccgccgtataagagccacc

SEQ ID NO: 271 - RNA, 71 nt, synthetic construct
  misc_feature 1..71: note = (CCG)8-8-UTR
  source 1..71: mol_type = other RNA
gggaaataagagagaaaagaagagtaagaagaaccgccgccgccgccgccgccgccgatataagagccacc

SEQ ID NO: 272 - RNA, 71 nt, synthetic construct
  misc_feature 1..71: note = (CCG)8-9-UTR
  source 1..71: mol_type = other RNA
gggaaataagagagaaaagaagagtaagaagaccgccgccgccgccgccgccgccgaatataagagccacc

SEQ ID NO: 273 - RNA, 71 nt, synthetic construct
  misc_feature 1..71: note = (CCG)8-10-UTR
  source 1..71: mol_type = other RNA
gggaaataagagagaaaagaagagtaagaagccgccgccgccgccgccgccgccgaaatataagagccacc

SEQ ID NO: 274 - RNA, 71 nt, synthetic construct
  misc_feature 1..71: note = (CCG)8-11-UTR
  source 1..71: mol_type = other RNA
gggaaataagagagaaaagaagagtaagaaccgccgccgccgccgccgccgccggaaatataagagccacc

SEQ ID NO: 275 - RNA, 71 nt, synthetic construct
  misc_feature 1..71: note = (CCG)8-12-UTR
  source 1..71: mol_type = other RNA
gggaaataagagagaaaagaagagtaagaccgccgccgccgccgccgccgccgagaaatataagagccacc

SEQ ID NO: 276 - RNA, 71 nt, synthetic construct
  misc_feature 1..71: note = (CCG)8-13-UTR
  source 1..71: mol_type = other RNA
gggaaataagagagaaaagaagagtaagccgccgccgccgccgccgccgccgaagaaatataagagccacc

SEQ ID NO: 277 - RNA, 71 nt, synthetic construct
  misc_feature 1..71: note = (CCG)8-14-UTR
  source 1..71: mol_type = other RNA
gggaaataagagagaaaagaagagtaaccgccgccgccgccgccgccgccggaagaaatataagagccacc

SEQ ID NO: 278 - RNA, 71 nt, synthetic construct
  misc_feature 1..71: note = (CCG)8-15-UTR
  source 1..71: mol_type = other RNA
gggaaataagagagaaaagaagagtaccgccgccgccgccgccgccgccgagaagaaatataagagccacc

SEQ ID NO: 279 - RNA, 71 nt, synthetic construct
  misc_feature 1..71: note = (CCG)8-16-UTR
  source 1..71: mol_type = other RNA
gggaaataagagagaaaagaagagtccgccgccgccgccgccgccgccgaagaagaaatataagagccacc

SEQ ID NO: 280 - RNA, 71 nt, synthetic construct
  misc_feature 1..71: note = (CCG)8-17-UTR
  source 1..71: mol_type = other RNA
gggaaataagagagaaaagaagagccgccgccgccgccgccgccgccgtaagaagaaatataagagccacc

SEQ ID NO: 281 - RNA, 71 nt, synthetic construct
  misc_feature 1..71: note = (CCG)8-18-UTR
  source 1..71: mol_type = other RNA
gggaaataagagagaaaagaagaccgccgccgccgccgccgccgccggtaagaagaaatataagagccacc

SEQ ID NO: 282 - RNA, 74 nt, synthetic construct
  misc_feature 1..74: note = (CCG)9-UTR
  source 1..74: mol_type = other RNA
gggaaataagagagaaaagaagagtaagaagaaatataagaccgccgccgccgccgccgccgccgccggccacc

SEQ ID NO: 283 - RNA, 74 nt, synthetic construct
  misc_feature 1..74: note = (CCG)9-1-UTR
  source 1..74: mol_type = other RNA
gggaaataagagagaaaagaagagtaagaagaaatataagccgccgccgccgccgccgccgccgccgagccacc

SEQ ID NO: 284 - RNA, 74 nt, synthetic construct
  misc_feature 1..74: note = (CCG)9-2-UTR
  source 1..74: mol_type = other RNA
gggaaataagagagaaaagaagagtaagaagaaatataaccgccgccgccgccgccgccgccgccggagccacc

SEQ ID NO: 285 - RNA, 74 nt, synthetic construct
  misc_feature 1..74: note = (CCG)9-3-UTR
  source 1..74: mol_type = other RNA
gggaaataagagagaaaagaagagtaagaagaaatataccgccgccgccgccgccgccgccgccgagagccacc

SEQ ID NO: 286 - RNA, 74 nt, synthetic construct
  misc_feature 1..74: note = (CCG)9-4-UTR
  source 1..74: mol_type = other RNA
gggaaataagagagaaaagaagagtaagaagaaatatccgccgccgccgccgccgccgccgccgaagagccacc

SEQ ID NO: 287 - RNA, 74 nt, synthetic construct
  misc_feature 1..74: note = (CCG)9-5-UTR
  source 1..74: mol_type = other RNA
gggaaataagagagaaaagaagagtaagaagaaataccgccgccgccgccgccgccgccgccgtaagagccacc

SEQ ID NO: 288 - RNA, 74 nt, synthetic construct
  misc_feature 1..74: note = (CCG)9-6-UTR
  source 1..74: mol_type = other RNA
gggaaataagagagaaaagaagagtaagaagaaatccgccgccgccgccgccgccgccgccgataagagccacc

SEQ ID NO: 289 - RNA, 74 nt, synthetic construct
  misc_feature 1..74: note = (CCG)9-7-UTR
  source 1..74: mol_type = other RNA
gggaaataagagagaaaagaagagtaagaagaaaccgccgccgccgccgccgccgccgccgtataagagccacc

SEQ ID NO: 290 - RNA, 74 nt, synthetic construct
  misc_feature 1..74: note = (CCG)9-8-UTR
  source 1..74: mol_type = other RNA
gggaaataagagagaaaagaagagtaagaagaaccgccgccgccgccgccgccgccgccgatataagagccacc

SEQ ID NO: 291 - RNA, 74 nt, synthetic construct
  misc_feature 1..74: note = (CCG)9-9-UTR
  source 1..74: mol_type = other RNA
gggaaataagagagaaaagaagagtaagaagaccgccgccgccgccgccgccgccgccgaatataagagccacc

SEQ ID NO: 292 - RNA, 74 nt, synthetic construct
  misc_feature 1..74: note = (CCG)9-10-UTR
  source 1..74: mol_type = other RNA
gggaaataagagagaaaagaagagtaagaagccgccgccgccgccgccgccgccgccgaaatataagagccacc

SEQ ID NO: 293 - RNA, 74 nt, synthetic construct
  misc_feature 1..74: note = (CCG)9-11-UTR
  source 1..74: mol_type = other RNA
gggaaataagagagaaaagaagagtaagaaccgccgccgccgccgccgccgccgccggaaatataagagccacc

SEQ ID NO: 294 - RNA, 74 nt, synthetic construct
  misc_feature 1..74: note = (CCG)9-12-UTR
  source 1..74: mol_type = other RNA
gggaaataagagagaaaagaagagtaagaccgccgccgccgccgccgccgccgccgagaaatataagagccacc

SEQ ID NO: 295 - RNA, 74 nt, synthetic construct
  misc_feature 1..74: note = (CCG)9-13-UTR
  source 1..74: mol_type = other RNA
gggaaataagagagaaaagaagagtaagccgccgccgccgccgccgccgccgccgaagaaatataagagccacc

SEQ ID NO: 296 - RNA, 74 nt, synthetic construct
  misc_feature 1..74: note = (CCG)9-14-UTR
  source 1..74: mol_type = other RNA
gggaaataagagagaaaagaagagtaaccgccgccgccgccgccgccgccgccggaagaaatataagagccacc

SEQ ID NO: 297 - RNA, 74 nt, synthetic construct
  misc_feature 1..74: note = (CCG)9-15-UTR
  source 1..74: mol_type = other RNA
gggaaataagagagaaaagaagagtaccgccgccgccgccgccgccgccgccgagaagaaatataagagccacc

SEQ ID NO: 298 - RNA, 74 nt, synthetic construct
  misc_feature 1..74: note = (CCG)9-16-UTR
  source 1..74: mol_type = other RNA
gggaaataagagagaaaagaagagtccgccgccgccgccgccgccgccgccgaagaagaaatataagagccacc

SEQ ID NO: 299 - RNA, 74 nt, synthetic construct
  misc_feature 1..74: note = (CCG)9-17-UTR
  source 1..74: mol_type = other RNA
gggaaataagagagaaaagaagagccgccgccgccgccgccgccgccgccgtaagaagaaatataagagccacc

SEQ ID NO: 300 - RNA, 74 nt, synthetic construct
  misc_feature 1..74: note = (CCG)9-18-UTR
  source 1..74: mol_type = other RNA
gggaaataagagagaaaagaagaccgccgccgccgccgccgccgccgccggtaagaagaaatataagagccacc

SEQ ID NO: 301 - RNA, 77 nt, synthetic construct
  misc_feature 1..77: note = (CCG)10-UTR
  source 1..77: mol_type = other RNA
gggaaataagagagaaaagaagagtaagaagaaatataagaccgccgccgccgccgccgccgccgccgccggccacc

SEQ ID NO: 302 - RNA, 77 nt, synthetic construct
  misc_feature 1..77: note = (CCG)10-1-UTR
  source 1..77: mol_type = other RNA
gggaaataagagagaaaagaagagtaagaagaaatataagccgccgccgccgccgccgccgccgccgccgagccacc

SEQ ID NO: 303 - RNA, 77 nt, synthetic construct
  misc_feature 1..77: note = (CCG)10-2-UTR
  source 1..77: mol_type = other RNA
gggaaataagagagaaaagaagagtaagaagaaatataaccgccgccgccgccgccgccgccgccgccggagccacc

SEQ ID NO: 304 - RNA, 77 nt, synthetic construct
  misc_feature 1..77: note = (CCG)10-3-UTR
  source 1..77: mol_type = other RNA
gggaaataagagagaaaagaagagtaagaagaaatataccgccgccgccgccgccgccgccgccgccgagagccacc

SEQ ID NO: 305 - RNA, 77 nt, synthetic construct
  misc_feature 1..77: note = (CCG)10-4-UTR
  source 1..77: mol_type = other RNA
gggaaataagagagaaaagaagagtaagaagaaatatccgccgccgccgccgccgccgccgccgccgaagagccacc

SEQ ID NO: 306 - RNA, 77 nt, synthetic construct
  misc_feature 1..77: note = (CCG)10-5-UTR
  source 1..77: mol_type = other RNA
gggaaataagagagaaaagaagagtaagaagaaataccgccgccgccgccgccgccgccgccgccgtaagagccacc

SEQ ID NO: 307 - RNA, 77 nt, synthetic construct
  misc_feature 1..77: note = (CCG)10-6-UTR
  source 1..77: mol_type = other RNA
gggaaataagagagaaaagaagagtaagaagaaatccgccgccgccgccgccgccgccgccgccgataagagccacc

SEQ ID NO: 308 - RNA, 77 nt, synthetic construct
  misc_feature 1..77: note = (CCG)10-7-UTR
  source 1..77: mol_type = other RNA
gggaaataagagagaaaagaagagtaagaagaaaccgccgccgccgccgccgccgccgccgccgtataagagccacc

SEQ ID NO: 309 - RNA, 77 nt, synthetic construct
  misc_feature 1..77: note = (CCG)10-8-UTR
  source 1..77: mol_type = other RNA
gggaaataagagagaaaagaagagtaagaagaaccgccgccgccgccgccgccgccgccgccgatataagagccacc

SEQ ID NO: 310 - RNA, 77 nt, synthetic construct
  misc_feature 1..77: note = (CCG)10-9-UTR
  source 1..77: mol_type = other RNA
gggaaataagagagaaaagaagagtaagaagaccgccgccgccgccgccgccgccgccgccgaatataagagccacc

SEQ ID NO: 311 - RNA, 77 nt, synthetic construct
  misc_feature 1..77: note = (CCG)10-10-UTR
  source 1..77: mol_type = other RNA
gggaaataagagagaaaagaagagtaagaagccgccgccgccgccgccgccgccgccgccgaaatataagagccacc

SEQ ID NO: 312 - RNA, 77 nt, synthetic construct
  misc_feature 1..77: note = (CCG)10-11-UTR
  source 1..77: mol_type = other RNA
gggaaataagagagaaaagaagagtaagaaccgccgccgccgccgccgccgccgccgccggaaatataagagccacc

SEQ ID NO: 313 - RNA, 77 nt, synthetic construct
  misc_feature 1..77: note = (CCG)10-12-UTR
  source 1..77: mol_type = other RNA
gggaaataagagagaaaagaagagtaagaccgccgccgccgccgccgccgccgccgccgagaaatataagagccacc

SEQ ID NO: 314 - RNA, 77 nt, synthetic construct
  misc_feature 1..77: note = (CCG)10-13-UTR
  source 1..77: mol_type = other RNA
gggaaataagagagaaaagaagagtaagccgccgccgccgccgccgccgccgccgccgaagaaatataagagccacc

SEQ ID NO: 315 - RNA, 77 nt, synthetic construct
  misc_feature 1..77: note = (CCG)10-14-UTR
  source 1..77: mol_type = other RNA
gggaaataagagagaaaagaagagtaaccgccgccgccgccgccgccgccgccgccggaagaaatataagagccacc

SEQ ID NO: 316 - RNA, 77 nt, synthetic construct
  misc_feature 1..77: note = (CCG)10-15-UTR
  source 1..77: mol_type = other RNA
gggaaataagagagaaaagaagagtaccgccgccgccgccgccgccgccgccgccgagaagaaatataagagccacc

SEQ ID NO: 317 - RNA, 77 nt, synthetic construct
  misc_feature 1..77: note = (CCG)10-16-UTR
  source 1..77: mol_type = other RNA
gggaaataagagagaaaagaagagtccgccgccgccgccgccgccgccgccgccgaagaagaaatataagagccacc

SEQ ID NO: 318 - RNA, 77 nt, synthetic construct
  misc_feature 1..77: note = (CCG)10-17-UTR
  source 1..77: mol_type = other RNA
gggaaataagagagaaaagaagagccgccgccgccgccgccgccgccgccgccgtaagaagaaatataagagccacc

SEQ ID NO: 319 - RNA, 77 nt, synthetic construct
  misc_feature 1..77: note = (CCG)10-18-UTR
  source 1..77: mol_type = other RNA
gggaaataagagagaaaagaagaccgccgccgccgccgccgccgccgccgccggtaagaagaaatataagagccacc

SEQ ID NO: 320 - RNA, 56 nt, synthetic construct
  misc_feature 1..56: note = (GCC)3-UTR
  source 1..56: mol_type = other RNA
gggaaataagagagaaaagaagagtaagaagaaatataagagccgccgccgccacc

SEQ ID NO: 321 - RNA, 56 nt, synthetic construct
  misc_feature 1..56: note = (GCC)3-1-UTR
  source 1..56: mol_type = other RNA
gggaaataagagagaaaagaagagtaagaagaaatataaggccgccgccagccacc

SEQ ID NO: 322 - RNA, 56 nt, synthetic construct; identical to SEQ ID NO: 169
  misc_feature 1..56: note = (GCC)3-2-UTR
  source 1..56: mol_type = other RNA

SEQ ID NO: 323 - RNA, 56 nt, synthetic construct
  misc_feature 1..56: note = (GCC)3-3-UTR
  source 1..56: mol_type = other RNA
gggaaataagagagaaaagaagagtaagaagaaatatagccgccgccagagccacc

SEQ ID NO: 324 - RNA, 56 nt, synthetic construct
  misc_feature 1..56: note = (GCC)3-4-UTR
  source 1..56: mol_type = other RNA
gggaaataagagagaaaagaagagtaagaagaaatatgccgccgccaagagccacc

SEQ ID NO: 325 - RNA, 56 nt, synthetic construct
  misc_feature 1..56: note = (GCC)3-5-UTR
  source 1..56: mol_type = other RNA
gggaaataagagagaaaagaagagtaagaagaaatagccgccgcctaagagccacc

SEQ ID NO: 326 - RNA, 56 nt, synthetic construct
  misc_feature 1..56: note = (GCC)3-6-UTR
  source 1..56: mol_type = other RNA
gggaaataagagagaaaagaagagtaagaagaaatgccgccgccataagagccacc

SEQ ID NO: 327 - RNA, 56 nt, synthetic construct
  misc_feature 1..56: note = (GCC)3-7-UTR
  source 1..56: mol_type = other RNA
gggaaataagagagaaaagaagagtaagaagaaagccgccgcctataagagccacc

SEQ ID NO: 328 - RNA, 56 nt, synthetic construct
  misc_feature 1..56: note = (GCC)3-8-UTR
  source 1..56: mol_type = other RNA
gggaaataagagagaaaagaagagtaagaagaagccgccgccatataagagccacc

SEQ ID NO: 329 - RNA, 56 nt, synthetic construct
  misc_feature 1..56: note = (GCC)3-9-UTR
  source 1..56: mol_type = other RNA
gggaaataagagagaaaagaagagtaagaagagccgccgccaatataagagccacc

SEQ ID NO: 330 - RNA, 56 nt, synthetic construct
  misc_feature 1..56: note = (GCC)3-10-UTR
  source 1..56: mol_type = other RNA
gggaaataagagagaaaagaagagtaagaaggccgccgccaaatataagagccacc

SEQ ID NO: 331 - RNA, 56 nt, synthetic construct; identical to SEQ ID NO: 178
  misc_feature 1..56: note = (GCC)3-11-UTR
  source 1..56: mol_type = other RNA

SEQ ID NO: 332 - RNA, 56 nt, synthetic construct
  misc_feature 1..56: note = (GCC)3-12-UTR
  source 1..56: mol_type = other RNA
gggaaataagagagaaaagaagagtaagagccgccgccagaaatataagagccacc

SEQ ID NO: 333 - RNA, 56 nt, synthetic construct
  misc_feature 1..56: note = (GCC)3-13-UTR
  source 1..56: mol_type = other RNA
gggaaataagagagaaaagaagagtaaggccgccgccaagaaatataagagccacc

SEQ ID NO: 334 - RNA, 56 nt, synthetic construct; identical to SEQ ID NO: 181
  misc_feature 1..56: note = (GCC)3-14-UTR
  source 1..56: mol_type = other RNA

SEQ ID NO: 335 - RNA, 56 nt, synthetic construct
  misc_feature 1..56: note = (GCC)3-15-UTR
  source 1..56: mol_type = other RNA
gggaaataagagagaaaagaagagtagccgccgccagaagaaatataagagccacc

SEQ ID NO: 336 - RNA, 56 nt, synthetic construct
  misc_feature 1..56: note = (GCC)3-16-UTR
  source 1..56: mol_type = other RNA
gggaaataagagagaaaagaagagtgccgccgccaagaagaaatataagagccacc

SEQ ID NO: 337 - RNA, 56 nt, synthetic construct
  misc_feature 1..56: note = (GCC)3-17-UTR
  source 1..56: mol_type = other RNA
gggaaataagagagaaaagaagaggccgccgcctaagaagaaatataagagccacc

SEQ ID NO: 338 - RNA, 56 nt, synthetic construct; identical to SEQ ID NO: 185
  misc_feature 1..56: note = (GCC)3-18-UTR
  source 1..56: mol_type = other RNA

SEQ ID NO: 339 - RNA, 59 nt, synthetic construct
  misc_feature 1..59: note = (GCC)4-UTR
  source 1..59: mol_type = other RNA
gggaaataagagagaaaagaagagtaagaagaaatataagagccgccgccgccgccacc

SEQ ID NO: 340 - RNA, 59 nt, synthetic construct
  misc_feature 1..59: note = (GCC)4-1-UTR
  source 1..59: mol_type = other RNA
gggaaataagagagaaaagaagagtaagaagaaatataaggccgccgccgccagccacc

SEQ ID NO: 341 - RNA, 59 nt, synthetic construct; identical to SEQ ID NO: 188
  misc_feature 1..59: note = (GCC)4-2-UTR
  source 1..59: mol_type = other RNA

SEQ ID NO: 342 - RNA, 59 nt, synthetic construct
  misc_feature 1..59: note = (GCC)4-3-UTR
  source 1..59: mol_type = other RNA
gggaaataagagagaaaagaagagtaagaagaaatatagccgccgccgccagagccacc

SEQ ID NO: 343 - RNA, 59 nt, synthetic construct
  misc_feature 1..59: note = (GCC)4-4-UTR
  source 1..59: mol_type = other RNA
gggaaataagagagaaaagaagagtaagaagaaatatgccgccgccgccaagagccacc

SEQ ID NO: 344 - RNA, 59 nt, synthetic construct
  misc_feature 1..59: note = (GCC)4-5-UTR
  source 1..59: mol_type = other RNA
gggaaataagagagaaaagaagagtaagaagaaatagccgccgccgcctaagagccacc

SEQ ID NO: 345 - RNA, 59 nt, synthetic construct
  misc_feature 1..59: note = (GCC)4-6-UTR
  source 1..59: mol_type = other RNA
gggaaataagagagaaaagaagagtaagaagaaatgccgccgccgccataagagccacc

SEQ ID NO: 346 - RNA, 59 nt, synthetic construct
  misc_feature 1..59: note = (GCC)4-7-UTR
  source 1..59: mol_type = other RNA
gggaaataagagagaaaagaagagtaagaagaaagccgccgccgcctataagagccacc

SEQ ID NO: 347 - RNA, 59 nt, synthetic construct
  misc_feature 1..59: note = (GCC)4-8-UTR
  source 1..59: mol_type = other RNA
gggaaataagagagaaaagaagagtaagaagaagccgccgccgccatataagagccacc

SEQ ID NO: 348 - RNA, 59 nt, synthetic construct
  misc_feature 1..59: note = (GCC)4-9-UTR
  source 1..59: mol_type = other RNA
gggaaataagagagaaaagaagagtaagaagagccgccgccgccaatataagagccacc

SEQ ID NO: 349 - RNA, 59 nt, synthetic construct
  misc_feature 1..59: note = (GCC)4-10-UTR
  source 1..59: mol_type = other RNA
gggaaataagagagaaaagaagagtaagaaggccgccgccgccaaatataagagccacc

SEQ ID NO: 350 - RNA, 59 nt, synthetic construct; identical to SEQ ID NO: 197
  misc_feature 1..59: note = (GCC)4-11-UTR
  source 1..59: mol_type = other RNA

SEQ ID NO: 351 - RNA, 59 nt, synthetic construct
  misc_feature 1..59: note = (GCC)4-12-UTR
  source 1..59: mol_type = other RNA
gggaaataagagagaaaagaagagtaagagccgccgccgccagaaatataagagccacc

SEQ ID NO: 352 - RNA, 59 nt, synthetic construct
  misc_feature 1..59: note = (GCC)4-13-UTR
  source 1..59: mol_type = other RNA
gggaaataagagagaaaagaagagtaaggccgccgccgccaagaaatataagagccacc

SEQ ID NO: 353 - RNA, 59 nt, synthetic construct; identical to SEQ ID NO: 200
  misc_feature 1..59: note = (GCC)4-14-UTR
  source 1..59: mol_type = other RNA

SEQ ID NO: 354 - RNA, 59 nt, synthetic construct
  misc_feature 1..59: note = (GCC)4-15-UTR
  source 1..59: mol_type = other RNA
gggaaataagagagaaaagaagagtagccgccgccgccagaagaaatataagagccacc

SEQ ID NO: 355 - RNA, 59 nt, synthetic construct
  misc_feature 1..59: note = (GCC)4-16-UTR
  source 1..59: mol_type = other RNA
gggaaataagagagaaaagaagagtgccgccgccgccaagaagaaatataagagccacc

SEQ ID NO: 356 - RNA, 59 nt, synthetic construct
  misc_feature 1..59: note = (GCC)4-17-UTR
  source 1..59: mol_type = other RNA
gggaaataagagagaaaagaagaggccgccgccgcctaagaagaaatataagagccacc

SEQ ID NO: 357 - RNA, 59 nt, synthetic construct; identical to SEQ ID NO: 204
  misc_feature 1..59: note = (GCC)4-18-UTR
  source 1..59: mol_type = other RNA

SEQ ID NO: 358 - RNA, 62 nt, synthetic construct
  misc_feature 1..62: note = (GCC)5-UTR
  source 1..62: mol_type = other RNA
gggaaataagagagaaaagaagagtaagaagaaatataagagccgccgccgccgccgccacc

SEQ ID NO: 359 - RNA, 62 nt, synthetic construct
  misc_feature 1..62: note = (GCC)5-1-UTR
  source 1..62: mol_type = other RNA
gggaaataagagagaaaagaagagtaagaagaaatataaggccgccgccgccgccagccacc

SEQ ID NO: 360 - RNA, 62 nt, synthetic construct; identical to SEQ ID NO: 207
  misc_feature 1..62: note = (GCC)5-2-UTR
  source 1..62: mol_type = other RNA

SEQ ID NO: 361 - RNA, 62 nt, synthetic construct
  misc_feature 1..62: note = (GCC)5-3-UTR
  source 1..62: mol_type = other RNA
gggaaataagagagaaaagaagagtaagaagaaatatagccgccgccgccgccagagccacc

SEQ ID NO: 362 - RNA, 62 nt, synthetic construct
  misc_feature 1..62: note = (GCC)5-4-UTR
  source 1..62: mol_type = other RNA
gggaaataagagagaaaagaagagtaagaagaaatatgccgccgccgccgccaagagccacc

SEQ ID NO: 363 - RNA, 62 nt, synthetic construct
  misc_feature 1..62: note = (GCC)5-5-UTR
  source 1..62: mol_type = other RNA
gggaaataagagagaaaagaagagtaagaagaaatagccgccgccgccgcctaagagccacc

SEQ ID NO: 364 - RNA, 62 nt, synthetic construct
  misc_feature 1..62: note = (GCC)5-6-UTR
  source 1..62: mol_type = other RNA
gggaaataagagagaaaagaagagtaagaagaaatgccgccgccgccgccataagagccacc

SEQ ID NO: 365 - RNA, 62 nt, synthetic construct
  misc_feature 1..62: note = (GCC)5-7-UTR
  source 1..62: mol_type = other RNA
gggaaataagagagaaaagaagagtaagaagaaagccgccgccgccgcctataagagccacc

SEQ ID NO: 366 - RNA, 62 nt, synthetic construct
  misc_feature 1..62: note = (GCC)5-8-UTR
  source 1..62: mol_type = other RNA
gggaaataagagagaaaagaagagtaagaagaagccgccgccgccgccatataagagccacc

SEQ ID NO: 367 - RNA, 62 nt, synthetic construct
  misc_feature 1..62: note = (GCC)5-9-UTR
  source 1..62: mol_type = other RNA
gggaaataagagagaaaagaagagtaagaagagccgccgccgccgccaatataagagccacc

SEQ ID NO: 368 - RNA, 62 nt, synthetic construct
  misc_feature 1..62: note = (GCC)5-10-UTR
  source 1..62: mol_type = other RNA
gggaaataagagagaaaagaagagtaagaaggccgccgccgccgccaaatataagagccacc

SEQ ID NO: 369 - RNA, 62 nt, synthetic construct; identical to SEQ ID NO: 216
  misc_feature 1..62: note = (GCC)5-11-UTR
  source 1..62: mol_type = other RNA

SEQ ID NO: 370 - RNA, 62 nt, synthetic construct
  misc_feature 1..62: note = (GCC)5-12-UTR
  source 1..62: mol_type = other RNA
gggaaataagagagaaaagaagagtaagagccgccgccgccgccagaaatataagagccacc

SEQ ID NO: 371 - RNA, 62 nt, synthetic construct
  misc_feature 1..62: note = (GCC)5-13-UTR
  source 1..62: mol_type = other RNA
gggaaataagagagaaaagaagagtaaggccgccgccgccgccaagaaatataagagccacc

SEQ ID NO: 372 - RNA, 62 nt, synthetic construct; identical to SEQ ID NO: 219
  misc_feature 1..62: note = (GCC)5-14-UTR
  source 1..62: mol_type = other RNA

SEQ ID NO: 373 - RNA, 62 nt, synthetic construct
  misc_feature 1..62: note = (GCC)5-15-UTR
  source 1..62: mol_type = other RNA
gggaaataagagagaaaagaagagtagccgccgccgccgccagaagaaatataagagccacc

SEQ ID NO: 374 - RNA, 62 nt, synthetic construct
  misc_feature 1..62: note = (GCC)5-16-UTR
  source 1..62: mol_type = other RNA
gggaaataagagagaaaagaagagtgccgccgccgccgccaagaagaaatataagagccacc

SEQ ID NO: 375 - RNA, 62 nt, synthetic construct
  misc_feature 1..62: note = (GCC)5-17-UTR
  source 1..62: mol_type = other RNA
gggaaataagagagaaaagaagaggccgccgccgccgcctaagaagaaatataagagccacc

SEQ ID NO: 376 - RNA, 62 nt, synthetic construct; identical to SEQ ID NO: 223
  misc_feature 1..62: note = (GCC)5-18-UTR
  source 1..62: mol_type = other RNA

SEQ ID NO: 377 - RNA, 65 nt, synthetic construct
  misc_feature 1..65: note = (GCC)6-UTR
  source 1..65: mol_type = other RNA
gggaaataagagagaaaagaagagtaagaagaaatataagagccgccgccgccgccgccgccacc

SEQ ID NO: 378 - RNA, 65 nt, synthetic construct
  misc_feature 1..65: note = (GCC)6-1-UTR
  source 1..65: mol_type = other RNA
gggaaataagagagaaaagaagagtaagaagaaatataaggccgccgccgccgccgccagccacc

SEQ ID NO: 379 - RNA, 65 nt, synthetic construct; identical to SEQ ID NO: 226
  misc_feature 1..65: note = (GCC)6-2-UTR
  source 1..65: mol_type = other RNA

SEQ ID NO: 380 - RNA, 65 nt, synthetic construct
  misc_feature 1..65: note = (GCC)6-3-UTR
  source 1..65: mol_type = other RNA
gggaaataagagagaaaagaagagtaagaagaaatatagccgccgccgccgccgccagagccacc

SEQ ID NO: 381 - RNA, 65 nt, synthetic construct
  misc_feature 1..65: note = (GCC)6-4-UTR
  source 1..65: mol_type = other RNA
gggaaataagagagaaaagaagagtaagaagaaatatgccgccgccgccgccgccaagagccacc

SEQ ID NO: 382 - RNA, 65 nt, synthetic construct
  misc_feature 1..65: note = (GCC)6-5-UTR
  source 1..65: mol_type = other RNA
gggaaataagagagaaaagaagagtaagaagaaatagccgccgccgccgccgcctaagagccacc

SEQ ID NO: 383 - RNA, 65 nt, synthetic construct
  misc_feature 1..65: note = (GCC)6-6-UTR
  source 1..65: mol_type = other RNA
gggaaataagagagaaaagaagagtaagaagaaatgccgccgccgccgccgccataagagccacc

SEQ ID NO: 384 - RNA, 65 nt, synthetic construct
  misc_feature 1..65: note = (GCC)6-7-UTR
  source 1..65: mol_type = other RNA
gggaaataagagagaaaagaagagtaagaagaaagccgccgccgccgccgcctataagagccacc

SEQ ID NO: 385 - RNA, 65 nt, synthetic construct
  misc_feature 1..65: note = (GCC)6-8-UTR
  source 1..65: mol_type = other RNA
gggaaataagagagaaaagaagagtaagaagaagccgccgccgccgccgccatataagagccacc

SEQ ID NO: 386 - RNA, 65 nt, synthetic construct
  misc_feature 1..65: note = (GCC)6-9-UTR
  source 1..65: mol_type = other RNA
gggaaataagagagaaaagaagagtaagaagagccgccgccgccgccgccaatataagagccacc

SEQ ID NO: 387 - RNA, 65 nt, synthetic construct
  misc_feature 1..65: note = (GCC)6-10-UTR
  source 1..65: mol_type = other RNA
gggaaataagagagaaaagaagagtaagaaggccgccgccgccgccgccaaatataagagccacc

SEQ ID NO: 388 - RNA, 65 nt, synthetic construct; identical to SEQ ID NO: 235
  misc_feature 1..65: note = (GCC)6-11-UTR
  source 1..65: mol_type = other RNA

SEQ ID NO: 389 - RNA, 65 nt, synthetic construct
  misc_feature 1..65: note = (GCC)6-12-UTR
  source 1..65: mol_type = other RNA
gggaaataagagagaaaagaagagtaagagccgccgccgccgccgccagaaatataagagccacc

SEQ ID NO: 390 - RNA, 65 nt, synthetic construct
  misc_feature 1..65: note = (GCC)6-13-UTR
  source 1..65: mol_type = other RNA
gggaaataagagagaaaagaagagtaaggccgccgccgccgccgccaagaaatataagagccacc

SEQ ID NO: 391 - RNA, 65 nt, synthetic construct; identical to SEQ ID NO: 238
  misc_feature 1..65: note = (GCC)6-14-UTR
  source 1..65: mol_type = other RNA

SEQ ID NO: 392 - RNA, 65 nt, synthetic construct
  misc_feature 1..65: note = (GCC)6-15-UTR
  source 1..65: mol_type = other RNA
gggaaataagagagaaaagaagagtagccgccgccgccgccgccagaagaaatataagagccacc

SEQ ID NO: 393 - RNA, 65 nt, synthetic construct
  misc_feature 1..65: note = (GCC)6-16-UTR
  source 1..65: mol_type = other RNA
gggaaataagagagaaaagaagagtgccgccgccgccgccgccaagaagaaatataagagccacc

SEQ ID NO: 394 - RNA, 65 nt, synthetic construct
  misc_feature 1..65: note = (GCC)6-17-UTR
  source 1..65: mol_type = other RNA
gggaaataagagagaaaagaagaggccgccgccgccgccgcctaagaagaaatataagagccacc

SEQ ID NO: 395 - RNA, 65 nt, synthetic construct; identical to SEQ ID NO: 242
  misc_feature 1..65: note = (GCC)6-18-UTR
  source 1..65: mol_type = other RNA

SEQ ID NO: 396 - RNA, 68 nt, synthetic construct
  misc_feature 1..68: note = (GCC)7-UTR
  source 1..68: mol_type = other RNA
gggaaataagagagaaaagaagagtaagaagaaatataagagccgccgccgccgccgccgccgccacc

SEQ ID NO: 397 - RNA, 68 nt, synthetic construct
  misc_feature 1..68: note = (GCC)7-1-UTR
  source 1..68: mol_type = other RNA
gggaaataagagagaaaagaagagtaagaagaaatataaggccgccgccgccgccgccgccagccacc

SEQ ID NO: 398 - RNA, 68 nt, synthetic construct; identical to SEQ ID NO: 245
  misc_feature 1..68: note = (GCC)7-2-UTR
  source 1..68: mol_type = other RNA

SEQ ID NO: 399 - RNA, 68 nt, synthetic construct
  misc_feature 1..68: note = (GCC)7-3-UTR
  source 1..68: mol_type = other RNA
gggaaataagagagaaaagaagagtaagaagaaatatagccgccgccgccgccgccgccagagccacc

SEQ ID NO: 400 - RNA, 68 nt, synthetic construct
  misc_feature 1..68: note = (GCC)7-4-UTR
  source 1..68: mol_type = other RNA
gggaaataagagagaaaagaagagtaagaagaaatatgccgccgccgccgccgccgccaagagccacc

SEQ ID NO: 401 - RNA, 68 nt, synthetic construct
  misc_feature 1..68: note = (GCC)7-5-UTR
  source 1..68: mol_type = other RNA
gggaaataagagagaaaagaagagtaagaagaaatagccgccgccgccgccgccgcctaagagccacc

SEQ ID NO: 402 - RNA, 68 nt, synthetic construct
  misc_feature 1..68: note = (GCC)7-6-UTR
  source 1..68: mol_type = other RNA
gggaaataagagagaaaagaagagtaagaagaaatgccgccgccgccgccgccgccataagagccacc

SEQ ID NO: 403 - RNA, 68 nt, synthetic construct
  misc_feature 1..68: note = (GCC)7-7-UTR
  source 1..68: mol_type = other RNA
gggaaataagagagaaaagaagagtaagaagaaagccgccgccgccgccgccgcctataagagccacc

SEQ ID NO: 404 - RNA, 68 nt, synthetic construct
  misc_feature 1..68: note = (GCC)7-8-UTR
  source 1..68: mol_type = other RNA
gggaaataagagagaaaagaagagtaagaagaagccgccgccgccgccgccgccatataagagccacc

SEQ ID NO: 405 - RNA, 68 nt, synthetic construct
  misc_feature 1..68: note = (GCC)7-9-UTR
  source 1..68: mol_type = other RNA
gggaaataagagagaaaagaagagtaagaagagccgccgccgccgccgccgccaatataagagccacc

SEQ ID NO: 406 - RNA, 68 nt, synthetic construct
  misc_feature 1..68: note = (GCC)7-10-UTR
  source 1..68: mol_type = other RNA
gggaaataagagagaaaagaagagtaagaaggccgccgccgccgccgccgccaaatataagagccacc

SEQ ID NO: 407 - RNA, 68 nt, synthetic construct; identical to SEQ ID NO: 254
  misc_feature 1..68: note = (GCC)7-11-UTR
  source 1..68: mol_type = other RNA

SEQ ID NO: 408 - RNA, 68 nt, synthetic construct
  misc_feature 1..68: note = (GCC)7-12-UTR
  source 1..68: mol_type = other RNA
gggaaataagagagaaaagaagagtaagagccgccgccgccgccgccgccagaaatataagagccacc

SEQ ID NO: 409 - RNA, 68 nt, synthetic construct
  misc_feature 1..68: note = (GCC)7-13-UTR
  source 1..68: mol_type = other RNA
gggaaataagagagaaaagaagagtaaggccgccgccgccgccgccgccaagaaatataagagccacc

SEQ ID NO: 410 - RNA, 68 nt, synthetic construct; identical to SEQ ID NO: 257
  misc_feature 1..68: note = (GCC)7-14-UTR
  source 1..68: mol_type = other RNA

SEQ ID NO: 411 - RNA, 68 nt, synthetic construct
  misc_feature 1..68: note = (GCC)7-15-UTR
  source 1..68: mol_type = other RNA
gggaaataagagagaaaagaagagtagccgccgccgccgccgccgccagaagaaatataagagccacc

SEQ ID NO: 412 - RNA, 68 nt, synthetic construct
  misc_feature 1..68: note = (GCC)7-16-UTR
  source 1..68: mol_type = other RNA
gggaaataagagagaaaagaagagtgccgccgccgccgccgccgccaagaagaaatataagagccacc

SEQ ID NO: 413 - RNA, 68 nt, synthetic construct
  misc_feature 1..68: note = (GCC)7-17-UTR
  source 1..68: mol_type = other RNA
gggaaataagagagaaaagaagaggccgccgccgccgccgccgcctaagaagaaatataagagccacc

SEQ ID NO: 414 - RNA, 68 nt, synthetic construct; identical to SEQ ID NO: 261
  misc_feature 1..68: note = (GCC)7-18-UTR
  source 1..68: mol_type = other RNA

SEQ ID NO: 415 - RNA, 71 nt, synthetic construct
  misc_feature 1..71: note = (GCC)8-UTR
  source 1..71: mol_type = other RNA
gggaaataagagagaaaagaagagtaagaagaaatataagagccgccgccgccgccgccgccgccgccacc

SEQ ID NO: 416 - RNA, 71 nt, synthetic construct
  misc_feature 1..71: note = (GCC)8-1-UTR
  source 1..71: mol_type = other RNA
gggaaataagagagaaaagaagagtaagaagaaatataaggccgccgccgccgccgccgccgccagccacc

SEQ ID NO: 417 - RNA, 71 nt, synthetic construct; identical to SEQ ID NO: 264
  misc_feature 1..71: note = (GCC)8-2-UTR
  source 1..71: mol_type = other RNA

SEQ ID NO: 418 - RNA, 71 nt, synthetic construct
  misc_feature 1..71: note = (GCC)8-3-UTR
  source 1..71: mol_type = other RNA
gggaaataagagagaaaagaagagtaagaagaaatatagccgccgccgccgccgccgccgccagagccacc

SEQ ID NO: 419 - RNA, 71 nt, synthetic construct
  misc_feature 1..71: note = (GCC)8-4-UTR
  source 1..71: mol_type = other RNA
gggaaataagagagaaaagaagagtaagaagaaatatgccgccgccgccgccgccgccgccaagagccacc

SEQ ID NO: 420 - RNA, 71 nt, synthetic construct
  misc_feature 1..71: note = (GCC)8-5-UTR
  source 1..71: mol_type = other RNA
gggaaataagagagaaaagaagagtaagaagaaatagccgccgccgccgccgccgccgcctaagagccacc

SEQ ID NO: 421 - RNA, 71 nt, synthetic construct
  misc_feature 1..71: note = (GCC)8-6-UTR
  source 1..71: mol_type = other RNA
gggaaataagagagaaaagaagagtaagaagaaatgccgccgccgccgccgccgccgccataagagccacc

SEQ ID NO: 422 - RNA, 71 nt, synthetic construct
  misc_feature 1..71: note = (GCC)8-7-UTR
  source 1..71: mol_type = other RNA
gggaaataagagagaaaagaagagtaagaagaaagccgccgccgccgccgccgccgcctataagagccacc

SEQ ID NO: 423 - RNA, 71 nt, synthetic construct
  misc_feature 1..71: note = (GCC)8-8-UTR
  source 1..71: mol_type = other RNA
gggaaataagagagaaaagaagagtaagaagaagccgccgccgccgccgccgccgccatataagagccacc

SEQ ID NO: 424 - RNA, 71 nt, synthetic construct
  misc_feature 1..71: note = (GCC)8-9-UTR
  source 1..71: mol_type = other RNA
gggaaataagagagaaaagaagagtaagaagagccgccgccgccgccgccgccgccaatataagagccacc

SEQ ID NO: 425 - RNA, 71 nt, synthetic construct
  misc_feature 1..71: note = (GCC)8-10-UTR
  source 1..71: mol_type = other RNA
gggaaataagagagaaaagaagagtaagaaggccgccgccgccgccgccgccgccaaatataagagccacc

SEQ ID NO: 426 - RNA, 71 nt, synthetic construct; identical to SEQ ID NO: 273
  misc_feature 1..71: note = (GCC)8-11-UTR
  source 1..71: mol_type = other RNA

SEQ ID NO: 427 - RNA, 71 nt, synthetic construct
  misc_feature 1..71: note = (GCC)8-12-UTR
  source 1..71: mol_type = other RNA
gggaaataagagagaaaagaagagtaagagccgccgccgccgccgccgccgccagaaatataagagccacc

SEQ ID NO: 428 - RNA, 71 nt, synthetic construct
  misc_feature 1..71: note = (GCC)8-13-UTR
  source 1..71: mol_type = other RNA
gggaaataagagagaaaagaagagtaaggccgccgccgccgccgccgccgccaagaaatataagagccacc

SEQ ID NO: 429 - RNA, 71 nt, synthetic construct; identical to SEQ ID NO: 276
  misc_feature 1..71: note = (GCC)8-14-UTR
  source 1..71: mol_type = other RNA

SEQ ID NO: 430 - RNA, 71 nt, synthetic construct
  misc_feature 1..71: note = (GCC)8-15-UTR
  source 1..71: mol_type = other RNA
gggaaataagagagaaaagaagagtagccgccgccgccgccgccgccgccagaagaaatataagagccacc

SEQ ID NO: 431 - RNA, 71 nt, synthetic construct
  misc_feature 1..71: note = (GCC)8-16-UTR
  source 1..71: mol_type = other RNA
gggaaataagagagaaaagaagagtgccgccgccgccgccgccgccgccaagaagaaatataagagccacc

SEQ ID NO: 432 - RNA, 71 nt, synthetic construct
  misc_feature 1..71: note = (GCC)8-17-UTR
  source 1..71: mol_type = other RNA
gggaaataagagagaaaagaagaggccgccgccgccgccgccgccgcctaagaagaaatataagagccacc

SEQ ID NO: 433 - RNA, 71 nt, synthetic construct; identical to SEQ ID NO: 280
  misc_feature 1..71: note = (GCC)8-18-UTR
  source 1..71: mol_type = other RNA

SEQ ID NO: 434 - RNA, 74 nt, synthetic construct
  misc_feature 1..74: note = (GCC)9-UTR
  source 1..74: mol_type = other RNA
gggaaataagagagaaaagaagagtaagaagaaatataagagccgccgccgccgccgccgccgccgccgccacc

SEQ ID NO: 435 - RNA, 74 nt, synthetic construct
  misc_feature 1..74: note = (GCC)9-1-UTR
  source 1..74: mol_type = other RNA
gggaaataagagagaaaagaagagtaagaagaaatataaggccgccgccgccgccgccgccgccgccagccacc

SEQ ID NO: 436 - RNA, 74 nt, synthetic construct; identical to SEQ ID NO: 283
  misc_feature 1..74: note = (GCC)9-2-UTR
  source 1..74: mol_type = other RNA

SEQ ID NO: 437 - RNA, 74 nt, synthetic construct
  misc_feature 1..74: note = (GCC)9-3-UTR
  source 1..74: mol_type = other RNA
gggaaataagagagaaaagaagagtaagaagaaatatagccgccgccgccgccgccgccgccgccagagccacc

SEQ ID NO: 438 - RNA, 74 nt, synthetic construct
  misc_feature 1..74: note = (GCC)9-4-UTR
  source 1..74: mol_type = other RNA
gggaaataagagagaaaagaagagtaagaagaaatatgccgccgccgccgccgccgccgccgccaagagccacc

SEQ ID NO: 439 - RNA, 74 nt, synthetic construct
  misc_feature 1..74: note = (GCC)9-5-UTR
  source 1..74: mol_type = other RNA
gggaaataagagagaaaagaagagtaagaagaaatagccgccgccgccgccgccgccgccgcctaagagccacc

SEQ ID NO: 440 - RNA, 74 nt, synthetic construct
  misc_feature 1..74: note = (GCC)9-6-UTR
  source 1..74: mol_type = other RNA
gggaaataagagagaaaagaagagtaagaagaaatgccgccgccgccgccgccgccgccgccataagagccacc

SEQ ID NO: 441 - RNA, 74 nt, synthetic construct
  misc_feature 1..74: note = (GCC)9-7-UTR
  source 1..74: mol_type = other RNA
gggaaataagagagaaaagaagagtaagaagaaagccgccgccgccgccgccgccgccgcctataagagccacc

SEQ ID NO: 442 - RNA, 74 nt, synthetic construct
  misc_feature 1..74: note = (GCC)9-8-UTR
  source 1..74: mol_type = other RNA
gggaaataagagagaaaagaagagtaagaagaagccgccgccgccgccgccgccgccgccatataagagccacc

SEQ ID NO: 443 - RNA, 74 nt, synthetic construct
  misc_feature 1..74: note = (GCC)9-9-UTR
  source 1..74: mol_type = other RNA
gggaaataagagagaaaagaagagtaagaagagccgccgccgccgccgccgccgccgccaatataagagccacc

SEQ ID NO: 444 - RNA, 74 nt, synthetic construct
  misc_feature 1..74: note = (GCC)9-10-UTR
  source 1..74: mol_type = other RNA
gggaaataagagagaaaagaagagtaagaaggccgccgccgccgccgccgccgccgccaaatataagagccacc

SEQ ID NO: 445 - RNA, 74 nt, synthetic construct; identical to SEQ ID NO: 292
  misc_feature 1..74: note = (GCC)9-11-UTR
  source 1..74: mol_type = other RNA

SEQ ID NO: 446 - RNA, 74 nt, synthetic construct
  misc_feature 1..74: note = (GCC)9-12-UTR
  source 1..74: mol_type = other RNA
gggaaataagagagaaaagaagagtaagagccgccgccgccgccgccgccgccgccagaaatataagagccacc

SEQ ID NO: 447 - RNA, 74 nt, synthetic construct
  misc_feature 1..74: note = (GCC)9-13-UTR
  source 1..74: mol_type = other RNA
gggaaataagagagaaaagaagagtaaggccgccgccgccgccgccgccgccgccaagaaatataagagccacc

SEQ ID NO: 448 - RNA, 74 nt, synthetic construct; identical to SEQ ID NO: 295
  misc_feature 1..74: note = (GCC)9-14-UTR
  source 1..74: mol_type = other RNA

SEQ ID NO: 449 - RNA, 74 nt, synthetic construct
  misc_feature 1..74: note = (GCC)9-15-UTR
  source 1..74: mol_type = other RNA
gggaaataagagagaaaagaagagtagccgccgccgccgccgccgccgccgccagaagaaatataagagccacc

SEQ ID NO: 450 - RNA, 74 nt, synthetic construct
  misc_feature 1..74: note = (GCC)9-16-UTR
  source 1..74: mol_type = other RNA
gggaaataagagagaaaagaagagtgccgccgccgccgccgccgccgccgccaagaagaaatataagagccacc

SEQ ID NO: 451 - RNA, 74 nt, synthetic construct
  misc_feature 1..74: note = (GCC)9-17-UTR
  source 1..74: mol_type = other RNA
gggaaataagagagaaaagaagaggccgccgccgccgccgccgccgccgcctaagaagaaatataagagccacc

SEQ ID NO: 452 - RNA, 74 nt, synthetic construct; identical to SEQ ID NO: 299
  misc_feature 1..74: note = (GCC)9-18-UTR
  source 1..74: mol_type = other RNA

SEQ ID NO: 453 - RNA, 77 nt, synthetic construct
  misc_feature 1..77: note = (GCC)10-UTR
  source 1..77: mol_type = other RNA
gggaaataagagagaaaagaagagtaagaagaaatataagagccgccgccgccgccgccgccgccgccgccgccacc

SEQ ID NO: 454 - RNA, 77 nt, synthetic construct
  misc_feature 1..77: note = (GCC)10-1-UTR
  source 1..77: mol_type = other RNA
gggaaataagagagaaaagaagagtaagaagaaatataaggccgccgccgccgccgccgccgccgccgccagccacc

SEQ ID NO: 455 - RNA, 77 nt, synthetic construct; identical to SEQ ID NO: 302
  misc_feature 1..77: note = (GCC)10-2-UTR
  source 1..77: mol_type = other RNA

SEQ ID NO: 456 - RNA, 77 nt, synthetic construct
  misc_feature 1..77: note = (GCC)10-3-UTR
  source 1..77: mol_type = other RNA
gggaaataagagagaaaagaagagtaagaagaaatatagccgccgccgccgccgccgccgccgccgccagagccacc

SEQ ID NO: 457 - RNA, 77 nt, synthetic construct
  misc_feature 1..77: note = (GCC)10-4-UTR
  source 1..77: mol_type = other RNA
gggaaataagagagaaaagaagagtaagaagaaatatgccgccgccgccgccgccgccgccgccgccaagagccacc

SEQ ID NO: 458 - RNA, 77 nt, synthetic construct
  misc_feature 1..77: note = (GCC)10-5-UTR
  source 1..77: mol_type = other RNA
gggaaataagagagaaaagaagagtaagaagaaatagccgccgccgccgccgccgccgccgccgcctaagagccacc

SEQ ID NO: 459 - RNA, 77 nt, synthetic construct
  misc_feature 1..77: note = (GCC)10-6-UTR
  source 1..77: mol_type = other RNA
gggaaataagagagaaaagaagagtaagaagaaatgccgccgccgccgccgccgccgccgccgccataagagccacc

SEQ ID NO: 460 - RNA, 77 nt, synthetic construct
  misc_feature 1..77: note = (GCC)10-7-UTR
  source 1..77: mol_type = other RNA
gggaaataagagagaaaagaagagtaagaagaaagccgccgccgccgccgccgccgccgccgcctataagagccacc

SEQ ID NO: 461 - RNA, 77 nt, synthetic construct
  misc_feature 1..77: note = (GCC)10-8-UTR
  source 1..77: mol_type = other RNA
gggaaataagagagaaaagaagagtaagaagaagccgccgccgccgccgccgccgccgccgccatataagagccacc

SEQ ID NO: 462 - RNA, 77 nt, synthetic construct
  misc_feature 1..77: note = (GCC)10-9-UTR
  source 1..77: mol_type = other RNA
gggaaataagagagaaaagaagagtaagaagagccgccgccgccgccgccgccgccgccgccaatataagagccacc

SEQ ID NO: 463 - RNA, 77 nt, synthetic construct
  misc_feature 1..77: note = (GCC)10-10-UTR
  source 1..77: mol_type = other RNA
gggaaataagagagaaaagaagagtaagaaggccgccgccgccgccgccgccgccgccgccaaatataagagccacc

SEQ ID NO: 464 - RNA, 77 nt, synthetic construct; identical to SEQ ID NO: 311
  misc_feature 1..77: note = (GCC)10-11-UTR
  source 1..77: mol_type = other RNA

SEQ ID NO: 465 - RNA, 77 nt, synthetic construct
  misc_feature 1..77: note = (GCC)10-12-UTR
  source 1..77: mol_type = other RNA
gggaaataagagagaaaagaagagtaagagccgccgccgccgccgccgccgccgccgccagaaatataagagccacc

SEQ ID NO: 466 - RNA, 77 nt, synthetic construct
  misc_feature 1..77: note = (GCC)10-13-UTR
  source 1..77: mol_type = other RNA
gggaaataagagagaaaagaagagtaaggccgccgccgccgccgccgccgccgccgccaagaaatataagagccacc

SEQ ID NO: 467 - RNA, 77 nt, synthetic construct; identical to SEQ ID NO: 314
  misc_feature 1..77: note = (GCC)10-14-UTR
  source 1..77: mol_type = other RNA

SEQ ID NO: 468 - RNA, 77 nt, synthetic construct
  misc_feature 1..77: note = (GCC)10-15-UTR
  source 1..77: mol_type = other RNA
gggaaataagagagaaaagaagagtagccgccgccgccgccgccgccgccgccgccagaagaaatataagagccacc

SEQ ID NO: 469 - RNA, 77 nt, synthetic construct
  misc_feature 1..77: note = (GCC)10-16-UTR
  source 1..77: mol_type = other RNA
gggaaataagagagaaaagaagagtgccgccgccgccgccgccgccgccgccgccaagaagaaatataagagccacc

SEQ ID NO: 470 - RNA, 77 nt, synthetic construct
  misc_feature 1..77: note = (GCC)10-17-UTR
  source 1..77: mol_type = other RNA
gggaaataagagagaaaagaagaggccgccgccgccgccgccgccgccgccgcctaagaagaaatataagagccacc

SEQ ID NO: 471 - RNA, 77 nt, synthetic construct; identical to SEQ ID NO: 318
  misc_feature 1..77: note = (GCC)10-18-UTR
  source 1..77: mol_type = other RNA

SEQ ID NO: 472 - RNA, 15 nt, synthetic construct
  misc_feature 1..15: note = KT1-UTR
  source 1..15: mol_type = other RNA
gggcccgccgccaac

SEQ ID NO: 473 - RNA, 15 nt, synthetic construct
  misc_feature 1..15: note = KT2-UTR
  source 1..15: mol_type = other RNA
gggcccgccgccacc

SEQ ID NO: 474 - RNA, 15 nt, synthetic construct
  misc_feature 1..15: note = KT3-UTR
  source 1..15: mol_type = other RNA
gggcccgccgccgac

SEQ ID NO: 475 - RNA, 15 nt, synthetic construct
  misc_feature 1..15: note = KT4-UTR
  source 1..15: mol_type = other RNA
gggcccgccgccgcc

SEQ ID NO: 476 - RNA, 47 nt, synthetic construct; identical to SEQ ID NO: 33
  misc_feature 1..47: note = 5UTR-001, Upstream UTR
  source 1..47: mol_type = other RNA

SEQ ID NO: 477 - RNA, 47 nt, synthetic construct
  misc_feature 1..47: note = 5UTR-002, Upstream UTR
  source 1..47: mol_type = other RNA
gggagatcagagagaaaagaagagtaagaagaaatataagagccacc

SEQ ID NO: 478 - RNA, 145 nt, synthetic construct
  misc_feature 1..145: note = 5UTR-003, Upstream UTR
  source 1..145: mol_type = other RNA
ggaataaaagtctcaacacaacatatacaaaacaaacgaatctcaagcaatcaagcattctacttctattgcagcaatttaaatcatttcttttaaagcaaaagcaattttctgaaaattttcaccatttacgaacgatagcaac

SEQ ID NO: 479 - RNA, 42 nt, synthetic construct
  misc_feature 1..42: note = 5UTR-004, Upstream UTR
  source 1..42: mol_type = other RNA
gggagacaagcttggcattccggtactgttggtaaagccacc

SEQ ID NO: 480 - RNA, 47 nt, synthetic construct; identical to SEQ ID NO: 477
  misc_feature 1..47: note = 5UTR-005, Upstream UTR
  source 1..47: mol_type = other RNA

SEQ ID NO: 481 - RNA, 145 nt, synthetic construct; identical to SEQ ID NO: 478
  misc_feature 1..145: note = 5UTR-006, Upstream UTR
  source 1..145: mol_type = other RNA

SEQ ID NO: 482 - RNA, 42 nt, synthetic construct; identical to SEQ ID NO: 479
  misc_feature 1..42: note = 5UTR-007, Upstream UTR
  source 1..42: mol_type = other RNA

SEQ ID NO: 483 - RNA, 47 nt, synthetic construct
  misc_feature 1..47: note = 5UTR-008, Upstream UTR
  source 1..47: mol_type = other RNA
gggaattaacagagaaaagaagagtaagaagaaatataagagccacc

SEQ ID NO: 484 - RNA, 47 nt, synthetic construct
  misc_feature 1..47: note = 5UTR-009, Upstream UTR
  source 1..47: mol_type = other RNA
gggaaattagacagaaaagaagagtaagaagaaatataagagccacc

SEQ ID NO: 485 - RNA, 47 nt, synthetic construct
  misc_feature 1..47: note = 5UTR-010, Upstream UTR
  source 1..47: mol_type = other RNA
gggaaataagagagtaaagaacagtaagaagaaatataagagccacc

SEQ ID NO: 486 - RNA, 47 nt, synthetic construct
  misc_feature 1..47: note = 5UTR-011, Upstream UTR
  source 1..47: mol_type = other RNA
gggaaaaaagagagaaaagaagactaagaagaaatataagagccacc

SEQ ID NO: 487 - RNA, 47 nt, synthetic construct
  misc_feature 1..47: note = 5UTR-012, Upstream UTR
  source 1..47: mol_type = other RNA
gggaaataagagagaaaagaagagtaagaagatatataagagccacc

SEQ ID NO: 488 - RNA, 47 nt, synthetic construct
  misc_feature 1..47: note = 5UTR-013, Upstream UTR
  source 1..47: mol_type = other RNA
gggaaataagagacaaaacaagagtaagaagaaatataagagccacc

SEQ ID NO: 489 - RNA, 47 nt, synthetic construct
  misc_feature 1..47: note = 5UTR-014, Upstream UTR
  source 1..47: mol_type = other RNA
gggaaattagagagtaaagaacagtaagtagaattaaaagagccacc

SEQ ID NO: 490 - RNA, 47 nt, synthetic construct
  misc_feature 1..47: note = 5UTR-015, Upstream UTR
  source 1..47: mol_type = other RNA
gggaaataagagagaatagaagagtaagaagaaatataagagccacc

SEQ ID NO: 491 - RNA, 47 nt, synthetic construct
  misc_feature 1..47: note = 5UTR-016, Upstream UTR
  source 1..47: mol_type = other RNA
gggaaataagagagaaaagaagagtaagaagaaaattaagagccacc

SEQ ID NO: 492 - RNA, 47 nt, synthetic construct
  misc_feature 1..47: note = 5UTR-017, Upstream UTR
  source 1..47: mol_type = other RNA
gggaaataagagagaaaagaagagtaagaagaaatttaagagccacc

SEQ ID NO: 493 - RNA, 47 nt, synthetic construct; identical to SEQ ID NO: 33
  misc_feature 1..47: note = 5UTR-018, Upstream UTR
  source 1..47: mol_type = other RNA

SEQ ID NO: 494 - RNA, 92 nt, synthetic construct
  misc_feature 1..92: note = 5UTR-019, Upstream UTR
  source 1..92: mol_type = other RNA
tcaagcttttggaccctcgtacagaagctaatacgactcactatagggaaataagagagaaaagaagagtaagaagaaatataagagccacc

SEQ ID NO: 495 - RNA, 140 nt, synthetic construct
  misc_feature 1..140: note = 5UTR-020, Upstream UTR
  source 1..140: mol_type = other RNA
ggacagatcgcctggagacgccatccacgctgttttgacctccatagaagacaccgggaccgatccagcctccgcggccgggaacggtgcattggaacgcggattccccgtgccaagagtgactcaccgtccttgacacg

SEQ ID NO: 496 - RNA, 42 nt, synthetic construct
  misc_feature 1..42: note = 5UTR-021, Upstream UTR
  source 1..42: mol_type = other RNA
ggcgctgcctacggaggtggcagccatctccttctcggcatc

SEQ ID NO: 497 - RNA, 371 nt, synthetic construct
  misc_feature 1..371: note = 3UTR-001 - Creatine Kinase
  source 1..371: mol_type = other RNA
gcgcctgcccacctgccaccgactgctggaacccagccagtgggagggcctggcccaccagagtcctgctccctcactcctcgccccgccccctgtcccagagtcccacctgggggctctctccacccttctcagagttccagtttcaaccagagttccaaccaatgggctccatcctctggattctggccaatgaaatatctccctggcagggtcctcttcttttcccagagctccaccccaaccaggagctctagttaatggagagctcccagcacactcggagcttgtgctttgtctccacgcaaagcgataaataaaagcattggtggcctttggtctttgaataaagcctgagtaggaagtctaga

SEQ ID NO: 498 - RNA, 568 nt, synthetic construct
  misc_feature 1..568: note = 3UTR-002 - Myoglobin
  source 1..568: mol_type = other RNA
gcccctgccgctcccacccccacccatctgggccccgggttcaagagagagcggggtctgatctcgtgtagccatatagagtttgcttctgagtgtctgctttgtttagtagaggtgggcaggaggagctgaggggctggggctggggtgttgaagttggctttgcatgcccagcgatgcgcctccctgtgggatgtcatcaccctgggaaccgggagtggcccttggctcactgtgttctgcatggtttggatctgaattaattgtcctttcttctaaatcccaaccgaacttcttccaacctccaaactggctgtaaccccaaatccaagccattaactacacctgacagtagcaattgtctgattaatcactggccccttgaagacagcagaatgtccctttgcaatgaggaggagatctgggctgggcgggccagctggggaagcatttgactatctggaacttgtgtgtgcctcctcaggtatggcagtgactcacctggttttaataaaacaacctgcaacatctcatggtctttgaataaagcctgagtaggaagtctaga

SEQ ID NO: 499 - RNA, 289 nt, synthetic construct
  misc_feature 1..289: note = 3UTR-003 - alpha-actin
  source 1..289: mol_type = other RNA
acacactccacctccagcacgcgacttctcaggacgacgaatcttctcaatgggggggcggctgagctccagccaccccgcagtcactttctttgtaacaacttccgttgctgccatcgtaaactgacacagtgtttataacgtgtacatacattaacttattacctcattttgttatttttcgaaacaaagccctgtggaagaaaatggaaaacttgaagaagcattaaagtcattctgttaagctgcgtaaatggtctttgaataaagcctgagtaggaagtctaga

SEQ ID NO: 500 - RNA, 379 nt, synthetic construct
  misc_feature 1..379: note = 3UTR-004 - Albumin
  source 1..379: mol_type = other RNA
catcacatttaaaagcatctcagcctaccatgagaataagagaaagaaaatgaagatcaaaagcttattcatctgtttttctttttcgttggtgtaaagccaacaccctgtctaaaaaacataaatttctttaatcattttgcctcttttctctgtgcttcaattaataaaaaatggaaagaatctaatagagtggtacagcactgttatttttcaaagatgtgttgctatcctgaaaattctgtaggttctgtggaagttccagtgttctctcttattccacttcggtagaggatttctagtttcttgtgggctaattaaataaatcattaatactcttctaatggtctttgaataaagcctgagtaggaagtctaga

SEQ ID NO: 501 - RNA, 118 nt, synthetic construct
  misc_feature 1..118: note = 3UTR-005 - alpha-globin
  source 1..118: mol_type = other RNA
gctgccttctgcggggcttgccttctggccatgcccttcttctctcccttgcacctgtacctcttggtctttgaataaagcctgagtaggaaggcggccgctcgagcatgcatctaga

SEQ ID NO: 502 - RNA, 908 nt, synthetic construct
  misc_feature 1..908: note = 3UTR-006 - G-CSF
  source 1..908: mol_type = other RNA
gccaagccctccccatcccatgtatttatctctatttaatatttatgtctatttaagcctcatatttaaagacagggaagagcagaacggagccccaggcctctgtgtccttccctgcatttctgagtttcattctcctgcctgtagcagtgagaaaaagctcctgtcctcccatcccctggactgggaggtagataggtaaataccaagtatttattactatgactgctccccagccctggctctgcaatgggcactgggatgagccgctgtgagcccctggtcctgagggtccccacctgggacccttgagagtatcaggtctcccacgtgggagacaagaaatccctgtttaatatttaaacagcagtgttccccatctgggtccttgcacccctcactctggcctcagccgactgcacagcggcccctgcatccccttggctgtgaggcccctggacaagcagaggtggccagagctgggaggcatggccctggggtcccacgaatttgctggggaatctcgtttttcttcttaagacttttgggacatggtttgactcccgaacatcaccgacgcgtctcctgtttttctgggtggcctcgggacacctgccctgcccccacgagggtcaggactgtgactctttttagggccaggcaggtgcctggacatttgccttgctggacggggactggggatgtgggagggagcagacaggaggaatcatgtcaggcctgtgtgtgaaaggaagctccactgtcaccctccacctcttcaccccccactcaccagtgtcccctccactgtcacattgtaactgaacttcaggataataaagtgtttgcctccatggtctttgaataaagcctgagtaggaaggcggccgctcgagcatgcatctaga

SEQ ID NO: 503 - RNA, 835 nt, synthetic construct
  misc_feature 1..835: note = 3UTR-007 - Col1a2; collagen, type I, alpha 2
  source 1..835: mol_type = other RNA
actcaatctaaattaaaaaagaaagaaatttgaaaaaactttctctttgccatttcttcttcttcttttttaactgaaagctgaatccttccatttcttctgcacatctacttgcttaaattgtgggcaaaagagaaaaagaaggattgatcagagcattgtgcaatacagtttcattaactccttcccccgctcccccaaaaatttgaatttttttttcaacactcttacacctgttatggaaaatgtcaacctttgtaagaaaaccaaaataaaaattgaaaaataaaaaccataaacatttgcaccacttgtggcttttgaatatcttccacagagggaagtttaaaacccaaacttccaaaggtttaaactacctcaaaacactttcccatgagtgtgatccacattgttaggtgctgacctagacagagatgaactgaggtccttgttttgttttgttcataatacaaaggtgctaattaatagtatttcagatacttgaagaatgttgatggtgctagaagaatttgagaagaaatactcctgtattgagttgtatcgtgtggtgtattttttaaaaaatttgatttagcattcatattttccatcttattcccaattaaaagtatgcagattatttgcccaaatcttcttcagattcagcatttgttctttgccagtctcattttcatcttcttccatggttccacagaagctttgtttcttgggcaagcagaaaaattaaattgtacctattttgtatatgtgagatgtttaaataaattgtgaaaaaaatgaaataaagcatgtttggttttccaaaagaacatat

SEQ ID NO: 504 - RNA, 297 nt, synthetic construct
  misc_feature 1..297: note = 3UTR-008 - Col6a2; collagen, type VI, alpha 2
  source 1..297: mol_type = other RNA
cgccgccgcccgggccccgcagtcgagggtcgtgagcccaccccgtccatggtgctaagcgggcccgggtcccacacggccagcaccgctgctcactcggacgacgccctgggcctgcacctctccagctcctcccacggggtccccgtagccccggcccccgcccagccccaggtctccccaggccctccgcaggctgcccggcctccctccccctgcagccatcccaaggctcctgacctacctggcccctgagctctggagcaagccctgacccaataaaggctttgaacccat

SEQ ID NO: 505 - RNA, 602 nt, synthetic construct
  misc_feature 1..602: note = 3UTR-009 - RPN1; ribophorin I
  source 1..602: mol_type = other RNA
ggggctagagccctctccgcacagcgtggagacggggcaaggaggggggttattaggattggtggttttgttttgctttgtttaaagccgtgggaaaatggcacaactttacctctgtgggagatgcaacactgagagccaaggggtgggagttgggataatttttatataaaagaagtttttccactttgaattgctaaaagtggcatttttcctatgtgcagtcactcctctcatttctaaaatagggacgtggccaggcacggtggctcatgcctgtaatcccagcactttgggaggccgaggcaggcggctcacgaggtcaggagatcgagactatcctggctaacacggtaaaaccctgtctctactaaaagtacaaaaaattagctgggcgtggtggtgggcacctgtagtcccagctactcgggaggctgaggcaggagaaaggcatgaatccaagaggcagagcttgcagtgagctgagatcacgccattgcactccagcctgggcaacagtgttaagactctgtctcaaatataaataaataaataaataaataaataaataaataaaaataaagcgagatgttgccctcaaa

SEQ ID NO: 506 - RNA, 785 nt, synthetic construct
  misc_feature 1..785: note = 3UTR-010 - LRP1; low density lipoproteinreceptor-related protein 1
  source 1..785: mol_type = other RNA
ggccctgccccgtcggactgcccccagaaagcctcctgccccctgccagtgaagtccttcagtgagcccctccccagccagcccttccctggccccgccggatgtataaatgtaaaaatgaaggaattacattttatatgtgagcgagcaagccggcaagcgagcacagtattatttctccatcccctccctgcctgctccttggcacccccatgctgccttcagggagacaggcagggagggcttggggctgcacctcctaccctcccaccagaacgcaccccactgggagagctggtggtgcagccttcccctccctgtataagacactttgccaaggctctcccctctcgccccatccctgcttgcccgctcccacagcttcctgagggctaattctgggaagggagagttctttgctgcccctgtctggaagacgtggctctgggtgaggtaggcgggaaaggatggagtgttttagttcttgggggaggccaccccaaaccccagccccaactccaggggcacctatgagatggccatgctcaacccccctcccagacaggccctccctgtctccagggcccccaccgaggttcccagggctggagacttcctctggtaaacattcctccagcctcccctcccctggggacgccaaggaggtgggccacacccaggaagggaaagcgggcagccccgttttggggacgtgaacgttttaataatttttgctgaattcctttacaactaaataacacagatattgttataaataaaattgt

SEQ ID NO: 507 - RNA, 3001 nt, synthetic construct
  misc_feature 1..3001: note = 3UTR-011 - Nnt1; cardiotrophin-like cytokine factor 1
  source 1..3001: mol_type = other RNA
atattaaggatcaagctgttagctaataatgccacctctgcagttttgggaacaggcaaataaagtatcagtatacatggtgatgtacatctgtagcaaagctcttggagaaaatgaagactgaagaaagcaaagcaaaaactgtatagagagatttttcaaaagcagtaatccctcaattttaaaaaaggattgaaaattctaaatgtctttctgtgcatattttttgtgttaggaatcaaaagtattttataaaaggagaaagaacagcctcattttagatgtagtcctgttggattttttatgcctcctcagtaaccagaaatgttttaaaaaactaagtgtttaggatttcaagacaacattatacatggctctgaaatatctgacacaatgtaaacattgcaggcacctgcattttatgttttttttttcaacaaatgtgactaatttgaaacttttatgaacttctgagctgtccccttgcaattcaaccgcagtttgaattaatcatatcaaatcagttttaattttttaaattgtacttcagagtctatatttcaagggcacattttctcactactattttaatacattaaaggactaaataatctttcagagatgctggaaacaaatcatttgctttatatgtttcattagaataccaatgaaacatacaacttgaaaattagtaatagtatttttgaagatcccatttctaattggagatctctttaatttcgatcaacttataatgtgtagtactatattaagtgcacttgagtggaattcaacatttgactaataaaatgagttcatcatgttggcaagtgatgtggcaattatctctggtgacaaaagagtaaaatcaaatatttctgcctgttacaaatatcaaggaagacctgctactatgaaatagatgacattaatctgtcttcactgtttataatacggatggattttttttcaaatcagtgtgtgttttgaggtcttatgtaattgatgacatttgagagaaatggtggctttttttagctacctctttgttcatttaagcaccagtaaagatcatgtctttttatagaagtgtagattttctttgtgactttgctatcgtgcctaaagctctaaatataggtgaatgtgtgatgaatactcagattatttgtctctctatataattagtttggtactaagtttctcaaaaaattattaacacatgaaagacaatctctaaaccagaaaaagaagtagtacaaattttgttactgtaatgctcgcgtttagtgagtttaaaacacacagtatcttttggttttataatcagtttctattttgctgtgcctgagattaagatctgtgtatgtgtgtgtgtgtgtgtgtgcgtttgtgtgttaaagcagaaaagacttttttaaaagttttaagtgataaatgcaatttgttaattgatcttagatcactagtaaactcagggctgaattataccatgtatattctattagaagaaagtaaacaccatctttattcctgccctttttcttctctcaaagtagttgtagttatatctagaaagaagcaattttgatttcttgaaaaggtagttcctgcactcagtttaaactaaaaataatcatacttggattttatttatttttgtcatagtaaaaattttaatttatatatatttttatttagtattatcttattctttgctatttgccaatcctttgtcatcaattgtgttaaatgaattgaaaattcatgccctgttcattttattttactttattggttaggatatttaaaggatttttgtatatataatttcttaaattaatattccaaaaggttagtggacttagattataaattatggcaaaaatctaaaaacaacaaaaatgatttttatacattctatttcattattcctctttttccaataagtcatacaattggtagatatgacttattttatttttgtattattcactatatctttatgatatttaagtataaataattaaaaaaatttattgtaccttatagtctgtcaccaaaaaaaaaaaattatctgtaggtagtgaaatgctaatgttgatttgtctttaagggcttgttaactatcctttattttctcatttgtcttaaattaggagtttgtgtttaaattactcatctaagcaaaaaatgtatataaatcccattactgggtatatacccaaaggattataaatcatgctgctataaagacacatgcacacgtatgtttattgcagcactattcacaatagcaaagacttggaaccaacccaaatgtccatcaatgatagacttgattaagaaaatgtgcacatatacaccatggaatactatgcagccataaaaaaggatgagttcatgtcctttgtagggacatggataaagctggaaaccatcattctgagcaaactattgcaaggacagaaaaccaaacactgcatgttctcactcataggtgggaattgaacaatgagaacacttggacacaaggtggggaacaccacacaccagggcctgtcatggggtggggggagtggggagggatagcattaggagatatacctaatgtaaatgatgagttaatgggtgcagcacaccaacatggcacatgtatacatatgtagcaaacctgcacgttgtgcacatgtaccctagaacttaaagtataattaaaaaaaaaaagaaaacagaagctatttataaagaagttatttgctgaaataaatgtgatctttcccattaaaaaaataaagaaattttggggtaaaaaaacacaatatattgtattcttgaaaaattctaagagagtggatgtgaagtgttctcaccacaaaagtgataactaattgaggtaatgcacatattaattagaaagattttgtcattccacaatgtatatatacttaaaaatatgttatacacaataaatacatacattaaaaaataagtaaatgta

SEQ ID NO: 508 - RNA, 1037 nt, synthetic construct
  misc_feature 1..1037: note = 3UTR-012 - Col6a1; collagen, type VI, alpha 1
  source 1..1037: mol_type = other RNA
cccaccctgcacgccggcaccaaaccctgtcctcccacccctccccactcatcactaaacagagtaaaatgtgatgcgaattttcccgaccaacctgattcgctagattttttttaaggaaaagcttggaaagccaggacacaacgctgctgcctgctttgtgcagggtcctccggggctcagccctgagttggcatcacctgcgcagggccctctggggctcagccctgagctagtgtcacctgcacagggccctctgaggctcagccctgagctggcgtcacctgtgcagggccctctggggctcagccctgagctggcctcacctgggttccccaccccgggctctcctgccctgccctcctgcccgccctccctcctgcctgcgcagctccttccctaggcacctctgtgctgcatcccaccagcctgagcaagacgccctctcggggcctgtgccgcactagcctccctctcctctgtccccatagctggtttttcccaccaatcctcacctaacagttactttacaattaaactcaaagcaagctcttctcctcagcttggggcagccattggcctctgtctcgttttgggaaaccaaggtcaggaggccgttgcagacataaatctcggcgactcggccccgtctcctgagggtcctgctggtgaccggcctggaccttggccctacagccctggaggccgctgctgaccagcactgaccccgacctcagagagtactcgcaggggcgctggctgcactcaagaccctcgagattaacggtgctaaccccgtctgctcctccctcccgcagagactggggcctggactggacatgagagccccttggtgccacagagggctgtgtcttactagaaacaacgcaaacctctccttcctcagaatagtgatgtgttcgacgttttatcaaaggccccctttctatgttcatgttagttttgctccttctgtgtttttttctgaaccatatccatgttgctgacttttccaaataaaggttttcactcctctc

SEQ ID NO: 509 - RNA, 577 nt, synthetic construct
  misc_feature 1..577: note = 3UTR-013 - Calr; calreticulin
  source 1..577: mol_type = other RNA
agaggcctgcctccagggctggactgaggcctgagcgctcctgccgcagagctggccgcgccaaataatgtctctgtgagactcgagaactttcatttttttccaggctggttcggatttggggtggattttggttttgttcccctcctccactctcccccaccccctccccgcccttttttttttttttttttaaactggtattttatctttgattctccttcagccctcacccctggttctcatctttcttgatcaacatcttttcttgcctctgtccccttctctcatctcttagctcccctccaacctggggggcagtggtgtggagaagccacaggcctgagatttcatctgctctccttcctggagcccagaggagggcagcagaagggggtggtgtctccaaccccccagcactgaggaagaacggggctcttctcatttcacccctccctttctcccctgcccccaggactgggccacttctgggtggggcagtgggtcccagattggctcacactgagaatgtaagaactacaaacaaaatttctattaaattaaattttgtgtctcc

SEQ ID NO: 510 - RNA, 2212 nt, synthetic construct
  misc_feature 1..2212: note = 3UTR-014 - Colla1; collagen, type I, alpha 1
  source 1..2212: mol_type = other RNA
ctccctccatcccaacctggctccctcccacccaaccaactttccccccaacccggaaacagacaagcaacccaaactgaaccccctcaaaagccaaaaaatgggagacaatttcacatggactttggaaaatatttttttcctttgcattcatctctcaaacttagtttttatctttgaccaaccgaacatgaccaaaaaccaaaagtgcattcaaccttaccaaaaaaaaaaaaaaaaaaagaataaataaataactttttaaaaaaggaagcttggtccacttgcttgaagacccatgcgggggtaagtccctttctgcccgttgggcttatgaaaccccaatgctgccctttctgctcctttctccacaccccccttggggcctcccctccactccttcccaaatctgtctccccagaagacacaggaaacaatgtattgtctgcccagcaatcaaaggcaatgctcaaacacccaagtggcccccaccctcagcccgctcctgcccgcccagcacccccaggccctgggggacctggggttctcagactgccaaagaagccttgccatctggcgctcccatggctcttgcaacatctccccttcgtttttgagggggtcatgccgggggagccaccagcccctcactgggttcggaggagagtcaggaagggccacgacaaagcagaaacatcggatttggggaacgcgtgtcaatcccttgtgccgcagggctgggcgggagagactgttctgttccttgtgtaactgtgttgctgaaagactacctcgttcttgtcttgatgtgtcaccggggcaactgcctgggggcggggatgggggcagggtggaagcggctccccattttataccaaaggtgctacatctatgtgatgggtggggtggggagggaatcactggtgctatagaaattgagatgcccccccaggccagcaaatgttcctttttgttcaaagtctatttttattccttgatatttttctttttttttttttttttttgtggatggggacttgtgaatttttctaaaggtgctatttaacatgggaggagagcgtgtgcggctccagcccagcccgctgctcactttccaccctctctccacctgcctctggcttctcaggcctctgctctccgacctctctcctctgaaaccctcctccacagctgcagcccatcctcccggctccctcctagtctgtcctgcgtcctctgtccccgggtttcagagacaacttcccaaagcacaaagcagtttttccccctaggggtgggaggaagcaaaagactctgtacctattttgtatgtgtataataatttgagatgtttttaattattttgattgctggaataaagcatgtggaaatgacccaaacataatccgcagtggcctcctaatttccttctttggagttgggggaggggtagacatggggaaggggctttggggtgatgggcttgccttccattcctgccctttccctccccactattctcttctagatccctccataaccccactcccctttctctcacccttcttataccgcaaacctttctacttcctctttcattttctattcttgcaatttccttgcaccttttccaaatcctcttctcccctgcaataccatacaggcaatccacgtgcacaacacacacacacactcttcacatctggggttgtccaaacctcatacccactccccttcaagcccatccactctccaccccctggatgccctgcacttggtggcggtgggatgctcatggatactgggagggtgaggggagtggaacccgtgaggaggacctgggggcctctccttgaactgacatgaagggtcatctggcctctgctcccttctcacccacgctgacctcctgccgaaggagcaacgcaacaggagaggggtctgctgagcctggcgagggtctgggagggaccaggaggaaggcgtgctccctgctcgctgtcctggccctgggggagtgagggagacagacacctgggagagctgtggggaaggcactcgcaccgtgctcttgggaaggaaggagacctggccctgctcaccacggactgggtgcctcgacctcctgaatccccagaacacaacccccctgggctggggtggtctggggaaccatcgtgcccccgcctcccgcctactcctttttaagctt

SEQ ID NO: 511 - RNA, 729 nt, synthetic construct
  misc_feature 1..729: note = 3UTR-015 - Plod1; procollagen-lysine, 2-oxoglutarate5-dioxygenase 1
  source 1..729: mol_type = other RNA
ttggccaggcctgaccctcttggacctttcttctttgccgacaaccactgcccagcagcctctgggacctcggggtcccagggaacccagtccagcctcctggctgttgacttcccattgctcttggagccaccaatcaaagagattcaaagagattcctgcaggccagaggcggaacacacctttatggctggggctctccgtggtgttctggacccagcccctggagacaccattcacttttactgctttgtagtgactcgtgctctccaacctgtcttcctgaaaaaccaaggcccccttcccccacctcttccatggggtgagacttgagcagaacaggggcttccccaagttgcccagaaagactgtctgggtgagaagccatggccagagcttctcccaggcacaggtgttgcaccagggacttctgcttcaagttttggggtaaagacacctggatcagactccaagggctgccctgagtctgggacttctgcctccatggctggtcatgagagcaaaccgtagtcccctggagacagcgactccagagaacctcttgggagacagaagaggcatctgtgcacagctcgatcttctacttgcctgtggggaggggagtgacaggtccacacaccacactgggtcaccctgtcctggatgcctctgaagagagggacagaccgtcagaaactggagagtttctattaaaggtcatttaaacca

SEQ ID NO: 512 - RNA, 847 nt, synthetic construct
  misc_feature 1..847: note = 3UTR-016 - Nucb1; nucleobindin 1
  source 1..847: mol_type = other RNA
tcctccgggaccccagccctcaggattcctgatgctccaaggcgactgatgggcgctggatgaagtggcacagtcagcttccctgggggctggtgtcatgttgggctcctggggcgggggcacggcctggcatttcacgcattgctgccaccccaggtccacctgtctccactttcacagcctccaagtctgtggctcttcccttctgtcctccgaggggcttgccttctctcgtgtccagtgaggtgctcagtgatcggcttaacttagagaagcccgccccctccccttctccgtctgtcccaagagggtctgctctgagcctgcgttcctaggtggctcggcctcagctgcctgggttgtggccgccctagcatcctgtatgcccacagctactggaatccccgctgctgctccgggccaagcttctggttgattaatgagggcatggggtggtccctcaagaccttcccctaccttttgtggaaccagtgatgcctcaaagacagtgtcccctccacagctgggtgccaggggcaggggatcctcagtatagccggtgaaccctgataccaggagcctgggcctccctgaacccctggcttccagccatctcatcgccagcctcctcctggacctcttggcccccagccccttccccacacagccccagaagggtcccagagctgaccccactccaggacctaggcccagcccctcagcctcatctggagcccctgaagaccagtcccacccacctttctggcctcatctgacactgctccgcatcctgctgtgtgtcctgttccatgttccggttccatccaaatacactttctggaacaaa

SEQ ID NO: 513 - RNA, 110 nt, synthetic construct
  misc_feature 1..110: note = 3UTR-017 - alpha-globin
  source 1..110: mol_type = other RNA
gctggagcctcggtggccatgcttcttgccccttgggcctccccccagcccctcctccccttcctgcacccgtacccccgtggtctttgaataaagtctgagtgggcggc

SEQ ID NO: 514 - RNA, 116 nt, synthetic construct
  misc_feature 1..116: note = 3UTR-018 - Downstream UTR
  source 1..116: mol_type = other RNA
taataggctggagcctcggtggccatgcttcttgccccttgggcctccccccagcccctcctccccttcctgcacccgtacccccgtggtctttgaataaagtctgagtgggcggc

SEQ ID NO: 515 - RNA, 118 nt, synthetic construct
  misc_feature 1..118: note = 3UTR-019- Downstream UTR
  source 1..118: mol_type = other RNA
tgataataggctggagcctcggtggccatgcttcttgccccttgggcctccccccagcccctcctccccttcctgcacccgtaccccctggtctttgaataaagtctgagtgggcggc

SEQ ID NO: 516 - RNA, 138 nt, synthetic construct
  misc_feature 1..138: note = 3UTR-018 + miR-122-5p binding site
  source 1..138: mol_type = other RNA
taataggctggagcctcggtggccatgcttcttgccccttgggcctccccccagcccctcctccccttcctgcacccgtaccccccaaacaccattgtcacactccagtggtctttgaataaagtctgagtgggcggc

SEQ ID NO: 517 - RNA, 138 nt, synthetic construct
  misc_feature 1..138: note = 3UTR-018 + miR-122-3p binding site
  source 1..138: mol_type = other RNA
taataggctggagcctcggtggccatgcttcttgccccttgggcctccccccagcccctcctccccttcctgcacccgtaccccctatttagtgtgataatggcgttgtggtctttgaataaagtctgagtgggcggc

SEQ ID NO: 518 - RNA, 141 nt, synthetic construct
  misc_feature 1..141: note = 3UTR-019 + miR-122 binding site
  source 1..141: mol_type = other RNA
tgataataggctggagcctcggtggccatgcttcttgccccttgggcctccccccagcccctcctccccttcctgcacccgtaccccccaaacaccattgtcacactccagtggtctttgaataaagtctgagtgggcggc

SEQ ID NO: 519 - RNA, 87 nt, synthetic construct
  misc_feature 1..87: note = mmiR-142
  source 1..87: mol_type = other RNA
gacagtgcagtcacccataaagtagaaagcactactaacagcactggagggtgtagtgtttcctactttatggatgagtgtactgtg

SEQ ID NO: 520 - RNA, 23 nt, synthetic construct
  misc_feature 1..23: note = mmiR-142-3p
  source 1..23: mol_type = other RNA
tgtagtgtttcctactttatgga

SEQ ID NO: 521 - RNA, 23 nt, synthetic construct
  misc_feature 1..23: note = mmiR-142-3p binding site
  source 1..23: mol_type = other RNA
tccataaagtaggaaacactaca

SEQ ID NO: 522 - RNA, 21 nt, synthetic construct
  misc_feature 1..21: note = mmiR-142-5p
  source 1..21: mol_type = other RNA
cataaagtagaaagcactact

SEQ ID NO: 523 - RNA, 21 nt, synthetic construct
  misc_feature 1..21: note = mmiR-142-5p binding site
  source 1..21: mol_type = other RNA
agtagtgctttctactttatg

SEQ ID NO: 524 - RNA, 85 nt, synthetic construct
  misc_feature 1..85: note = miR-122
  source 1..85: mol_type = other RNA
ccttagcagagctgtggagtgtgacaatggtgtttgtgtctaaactatcaaacgccattatcacactaaatagctactgctaggc

SEQ ID NO: 525 - RNA, 22 nt, synthetic construct
  misc_feature 1..22: note = miR-122-3p
  source 1..22: mol_type = other RNA
aacgccattatcacactaaata

SEQ ID NO: 526 - RNA, 22 nt, synthetic construct
  misc_feature 1..22: note = miR-122-3p binding site
  source 1..22: mol_type = other RNA
tatttagtgtgataatggcgtt

SEQ ID NO: 527 - RNA, 22 nt, synthetic construct
  misc_feature 1..22: note = miR-122-5p
  source 1..22: mol_type = other RNA
tggagtgtgacaatggtgtttg

SEQ ID NO: 528 - RNA, 22 nt, synthetic construct
  misc_feature 1..22: note = miR-122-5p binding site
  source 1..22: mol_type = other RNA
caaacaccattgtcacactcca

SEQ ID NO: 529-530 - skipped (2 entries)

SEQ ID NO: 531 - RNA, 262 nt, synthetic construct
  misc_feature 1..262: note = Tubulin-like
  source 1..262: mol_type = other RNA
gtacaccggcatcgactaatcagggccaggctcgaggctttgtctccctaccgcgcgccgattctcccgcctcccagccccggcgcacgcgcgccccgcccagcctgctttccctccgcgccctcccctctcctttctccctctcagaaccttcctgccgtcgcgtttgcacctcgctgctccagcctctcgcattccaaccttccagcctgcgacctgcggagacttagccccatacataccttgaggcgagcttttaacc

SEQ ID NO: 532 - RNA, 57 nt, synthetic construct
  misc_feature 1..57: note = GC Scramble #1-UTR
  source 1..57: mol_type = other RNA
gggaaataagagagaaaagaagagtaagaagaaatataagaggggcgcccggccacc

SEQ ID NO: 533 - RNA, 57 nt, synthetic construct
  misc_feature 1..57: note = GC Scramble #2-UTR
  source 1..57: mol_type = other RNA
gggaaataagagagaaaagaagagtaagaagaaatataagagcccgcccgcgccacc

SEQ ID NO: 534 - RNA, 57 nt, synthetic construct
  misc_feature 1..57: note = GC Scramble #3-UTR
  source 1..57: mol_type = other RNA
gggaaataagagagaaaagaagagtaagaagaaatataagagcgccccgcggccacc

SEQ ID NO: 535 - RNA, 67 nt, synthetic construct; identical to SEQ ID NO: 73
  misc_feature 1..67: note = GC1-UTR
  source 1..67: mol_type = other RNA